European Patent Application EP 4 328 241 A2, published February 28, 2024. Title: MULTISPECIFIC MOLECULES COMPRISING A NON-IMMUNOGLOBULIN HETERODIMERIZATION DOMAIN AND USES THEREOF. Applicant: Marengo Therapeutics, Inc. Application EP. The sequence listing filed with the application follows.

SEQUENCE LISTING (171 sequences)

SEQ ID NO: 1 - protein, 93 aa, Homo sapiens
PDIQNPDPAVYQLRDSKSSDKSVCLFTDFDSQTNVSQSKDSDVYITDKCVLDMRSMDFKSNSAVAWSNKSDFACANAFNNSIIPEDTFFPSPE

SEQ ID NO: 2 - protein, 130 aa, Homo sapiens
EDLNKVFPPEVALFEPSEAEISHTQKATLVCLATGFYPDHVELSWWVNGKEVHSGVCTDPQPLKEQPALNDSRYALSSRLRVSATFWQDPRNHFRCQVQFYGLSEADEWTQARAKPVTQIVSAEAWGRAD

SEQ ID NO: 3-4 - skipped (2 entries)

SEQ ID NO: 5 - protein, 114 aa, Homo sapiens
NWVNVISDLKKIEDLIQSMHIDATLYTESDVHPSCKVTAMKCFLLELQVISLESGDASIHDTVENLIILANNSLSSNGNVTESGCKECEELEEKNIKEFLQSFVHIVQMFINTS

SEQ ID NO: 6 - protein, 77 aa, synthetic construct
  REGION 1..77: note = source = /note="Description of Artificial Sequence: Synthetic polypeptide"
MAPRRARGCRTLGLPALLLLLLLRPPATRGITCPPPMSVEHADIWVKSYSLYSRERYICNSGFKRKAGTSSLTECVL

SEQ ID NO: 7 - protein, 20 aa, synthetic construct
  REGION 1..20: note = source = /note="Description of Artificial Sequence: Synthetic peptide"
SGGSGGGGSGGGSGGGGSLQ

SEQ ID NO: 8 - protein, 133 aa, Homo sapiens [sequence omitted]

SEQ ID NO: 9 - protein, 157 aa, Homo sapiens
YFGKLESKLSVIRNLNDQVLFIDQGNRPLFEDMTDSDCRDNAPRTIFIISMYKDSQPRGMAVTISVKCEKISTLSCENKIISFKEMNPPDNIKDTKSDIIFFQRSVPGHDNKMQFESSSYEGYFLACEKERDLFKLILKKEDELGDRSIMFTVQNED

SEQ ID NO: 10 - protein, 133 aa, Homo sapiens [sequence omitted]

SEQ ID NO: 11 - protein, 138 aa, Homo sapiens
QDPYVKEAENLKKYFNAGHSDVADNGTLFLGILKNWKEESDRKIMQSQIVSFYFKLFKNFKDDQSIQKSVETIKEDMNVKFFNSNKKKRDDFEKLTNYSVTDLNVQRKAIHELIQVMAELSPAAKTGKRKRSQMLFRG

SEQ ID NO: 12 - protein, 454 aa, synthetic construct
  REGION 1..454: note = source = /note="Description of Artificial Sequence: Synthetic polypeptide"
METDTLLLWVLLLWVPGSTGQVQLVESGGGVVQPGRSLRLSCAASGFTFSSYTMHWVRQAPGKGLEWVTFISYDGNNKYYADSVKGRFTISRDNSKNTLYLQMNSLRAEDTAIYYCARTGWLGPFDYWGQGTLVTVSSASTKGPSVFPLAPSSKSTSGGTAALGCLVKDYFPEPVTVSWNSGALTSGVHTFPAVLQSSGLYSLSSVVTVPSSSLGTQTYICNVNHKPSNTKVDKRVEPKSCDKTHTCPPCPAPELLGGPSVFLFPPKPKDTLMISRTPEVTCVVVDVSHEDPEVKFNWYVDGVEVHNAKTKPREEQYNSTYRVVSVLTVLHQDWLNGKEYKCKVSNKALPAPIEKTISKAKPDIQNPDPAVYQLRDSKSSDKSVCLFTDFDSQTNVSQSKDSDVYITDKCVLDMRSMDFKSNSAVAWSNKSDFACANAFNNSIIPEDTFFPSPE

SEQ ID NO: 13 - protein, 488 aa, synthetic construct
  REGION 1..488: note = source = /note="Description of Artificial Sequence: Synthetic polypeptide"
METDTLLLWVLLLWVPGSTGQVQLVESGGGVVQPGRSLRLSCAASGFTFSSYGMHWVRQAPGKGLEWVAFIRYDGSNKYYADSVKGRFTISRDNSKNTLYLQMNSLRAEDTAVYYCKTHGSHDNWGQGTMVTVSSASTKGPSVFPLAPSSKSTSGGTAALGCLVKDYFPEPVTVSWNSGALTSGVHTFPAVLQSSGLYSLSSVVTVPSSSLGTQTYICNVNHKPSNTKVDKRVEPKSCDKTHTCPPCPAPELLGGPSVFLFPPKPKDTLMISRTPEVTCVVVDVSHEDPEVKFNWYVDGVEVHNAKTKPREEQYNSTYRVVSVLTVLHQDWLNGKEYKCKVSNKALPAPIEKTISKAKEDLNKVFPPEVALFEPSEAEISHTQKATLVCLATGFYPDHVELSWWVNGKEVHSGVCTDPQPLKEQPALNDSRYALSSRLRVSATFWQDPRNHFRCQVQFYGLSEADEWTQARAKPVTQIVSAEAWGRAD

SEQ ID NO: 14 - protein, 235 aa, synthetic construct
  REGION 1..235: note = source = /note="Description of Artificial Sequence: Synthetic polypeptide"
METDTLLLWVLLLWVPGSTGEIVLTQSPGTLSLSPGERATLSCRASQSVGSSYLAWYQQKPGQAPRLLIYGAFSRATGIPDRFSGSGSGTDFTLTISRLEPEDFAVYYCQQYGSSPWTFGQGTKVEIKRTVAAPSVFIFPPSDEQLKSGTASVVCLLNNFYPREAKVQWKVDNALQSGNSQESVTEQDSKDSTYSLSSTLTLSKADYEKHKVYACEVTHQGLSSPVTKSFNRGEC

SEQ ID NO: 15 - protein, 237 aa, synthetic construct
  REGION 1..237: note = source = /note="Description of Artificial Sequence: Synthetic polypeptide"
METDTLLLWVLLLWVPGSTGQSVLTQPPSVSGAPGQRVTISCSGSRSNIGSNTVKWYQQLPGTAPKLLIYYNDQRPSGVPDRFSGSKSGTSASLAITGLQAEDEADYYCQSYDRYTHPALLFGTGTKVTVLGQPKANPTVTLFPPSSEELQANKATLVCLISDFYPGAVTVAWKADGSPVKAGVETTKPSKQSNNKYAASSYLSLTPEQWKSHRSYSCQVTHEGSTVEKTVAPTECS

SEQ ID NO: 16 - DNA, 354 bp, synthetic construct
  misc_feature 1..354: note = source = /note="Description of Artificial Sequence: Synthetic polynucleotide"
  source 1..354: mol_type = other DNA
caggtgcagctggtggaatctggtggcggagttgtgcagcctggcagatccctgagactgtcttgtgccgcctccggcttcaccttctccagctacaccatgcactgggtccgacaggcccctggcaaaggattggagtgggtcaccttcatctcttacgacggcaacaacaagtactacgccgactccgtgaagggcagattcaccatctctcgggacaactccaagaacaccctgtacctgcagatgaactccctgagagccgaggacaccgccatctactactgtgctagaaccggctggctgggcccctttgattattggggacagggcaccctggtcaccgtgtcctct

SEQ ID NO: 17 - DNA, 324 bp, synthetic construct
  misc_feature 1..324: note = source = /note="Description of Artificial Sequence: Synthetic polynucleotide"
  source 1..324: mol_type = other DNA
gagatcgtgctgacccagtctcctggcacactgtcactgtctccaggcgagagagctaccctgtcctgtagagcctctcagtccgtgggctcctcttacctggcttggtatcagcagaagcccggccaggctcctagactgttgatctacggcgccttctccagagccacaggcatccctgatagattctccggctctggctctggcaccgacttcaccctgaccatctccagactggaacccgaggacttcgccgtgtactactgtcagcagtacggctcctctccttggacctttggccagggcaccaaggtggaaatcaag

SEQ ID NO: 18 - DNA, 345 bp, synthetic construct
  misc_feature 1..345: note = source = /note="Description of Artificial Sequence: Synthetic polynucleotide"
  source 1..345: mol_type = other DNA
caggtgcagctggtggaatctggtggcggagttgtgcagcctggcagatccctgagactgtcttgtgccgcctccggcttcaccttctcctcttacggaatgcactgggtccgacaggcccctggcaaaggattggagtgggtcgccttcatcagatacgacggctccaacaagtactacgccgactccgtgaagggcagattcaccatctctcgggacaactccaagaacaccctgtacctgcagatgaactccctgagagccgaggacaccgccgtgtactactgcaagacccacggctctcacgacaattggggccagggcacaatggtcaccgtgtcctct

SEQ ID NO: 19 - DNA, 333 bp, synthetic construct
  misc_feature 1..333: note = source = /note="Description of Artificial Sequence: Synthetic polynucleotide"
  source 1..333: mol_type = other DNA
cagtccgtgttgacccagcctccttctgtttctggcgctcctggccagagagtgaccatctcttgctccggctctcggtccaacatcggctccaataccgtgaagtggtatcagcagctgcccggcacagctcccaaactgctgatctactacaacgaccagcggccttctggcgtgcccgatagattctctggctccaagtctggcacctctgccagcctggctattaccggactgcaggctgaggacgaggccgactactactgccagtcttacgaccggtacacccatcctgctctgctgtttggcaccggcaccaaagtgacagtgctg

SEQ ID NO: 20 - DNA, 321 bp, synthetic construct
  misc_feature 1..321: note = source = /note="Description of Artificial Sequence: Synthetic polynucleotide"
  source 1..321: mol_type = other DNA
cggacagtggccgctccttccgtgttcatcttcccaccttccgacgagcagctgaagtccggcacagcttctgtcgtgtgcctgctgaacaacttctaccctcgggaagccaaggtgcagtggaaggtggacaatgccctgcagtccggcaactcccaagagtctgtgaccgagcaggactccaaggacagcacctacagcctgtcctccacactgaccctgtccaaggccgactacgagaagcacaaggtgtacgcctgcgaagtgacccatcagggcctgtctagccctgtgaccaagtctttcaaccggggcgagtgc

SEQ ID NO: 21 - DNA, 318 bp, synthetic construct
  misc_feature 1..318: note = source = /note="Description of Artificial Sequence: Synthetic polynucleotide"
  source 1..318: mol_type = other DNA
ggccagcctaaggccaatcctaccgtgacactgttccctccatcctccgaagaactgcaggccaacaaggctaccctcgtgtgcctgatctccgacttttaccctggcgctgtgaccgtggcctggaaggctgatggatctcctgtgaaggctggcgtggaaaccaccaagccttccaagcagtccaacaacaaatacgccgcctcctcctacctgtctctgacccctgaacagtggaagtcccaccggtcctacagctgccaagtgacccatgagggctccaccgtggaaaagaccgtggctcctaccgagtgctcc

SEQ ID NO: 22 - DNA, 309 bp, synthetic construct
  misc_feature 1..309: note = source = /note="Description of Artificial Sequence: Synthetic polynucleotide"
  source 1..309: mol_type = other DNA
gcttccaccaagggaccctctgtgttccctctggctccttccagcaagtctacctctggcggaacagctgctctgggctgcctggtcaaggactactttcctgagcctgtgaccgtgtcttggaactctggcgctctgacatccggcgtgcacacctttccagctgtgctgcaatcctccggcctgtactctctgtcctccgtcgtgaccgtgccttctagctctctgggcacccagacctacatctgcaatgtgaaccacaagccttccaacaccaaggtggacaagagagtggaacccaagtcctgc

SEQ ID NO: 23 - DNA, 360 bp, synthetic construct
  misc_feature 1..360: note = source = /note="Description of Artificial Sequence: Synthetic polynucleotide"
  source 1..360: mol_type = other DNA
gataagacccacacctgtccaccatgtcctgctccagaactgctcggcggaccttccgtgttcctgtttcctccaaagcctaaggacaccctgatgatctctcggacccctgaagtgacctgcgtggtggtggatgtgtctcacgaggatcccgaagtgaagttcaattggtacgtggacggcgtggaagtgcacaacgccaagaccaagcctagagaggaacagtacaactccacctacagagtggtgtccgtgctgaccgtgctgcaccaggattggctgaacggcaaagagtacaagtgcaaggtgtccaacaaggccctgcctgctcctatcgaaaagaccatctccaaggccaaa

SEQ ID NO: 24 - DNA, 279 bp, synthetic construct
  misc_feature 1..279: note = source = /note="Description of Artificial Sequence: Synthetic polynucleotide"
  source 1..279: mol_type = other DNA
cctgacattcagaaccccgatcctgccgtgtaccagctgagagactccaagtcctccgataagtctgtgtgcctgttcaccgacttcgactcccagaccaacgtgtcccagtccaaggactccgacgtgtacatcaccgataagtgcgtgctggacatgcggagcatggacttcaagtctaactccgccgtggcctggtctaacaagtccgatttcgcctgcgccaacgccttcaacaacagcattatccccgaggacacattcttcccatcacctgag

SEQ ID NO: 25 - DNA, 390 bp, synthetic construct
  misc_feature 1..390: note = source = /note="Description of Artificial Sequence: Synthetic polynucleotide"
  source 1..390: mol_type = other DNA
gaggacctgaacaaggttttcccacctgaggtggccctgttcgagccttctgaggctgagatctctcacacccagaaagctaccctcgtgtgtctggccaccggcttctaccctgatcacgtggaactgtcttggtgggtcaacggaaaagaggtgcactccggcgtctgcaccgatcctcagcctctgaaagaacagcccgctctgaacgactccagatacgccctgtcctctcggctgagagtgtctgccaccttctggcaggaccctcggaaccactttagatgccaggtgcagttctacggcctgtccgaggctgatgagtggacccaggctagagccaagccagtgacacagatcgtgtctgccgaagcctggggcagagccgat

SEQ ID NO: 26-28 - skipped (3 entries)

SEQ ID NO: 29 - DNA, 12 bp, synthetic construct
  misc_feature 1..12: note = source = /note="Description of Artificial Sequence: Synthetic oligonucleotide"
  source 1..12: mol_type = other DNA
ggtggcggagga

SEQ ID NO: 30 - DNA, 15 bp, synthetic construct
  misc_feature 1..15: note = source = /note="Description of Artificial Sequence: Synthetic oligonucleotide"
  source 1..15: mol_type = other DNA
ggtggcggaggaagc

SEQ ID NO: 31 - DNA, 18 bp, synthetic construct
  misc_feature 1..18: note = source = /note="Description of Artificial Sequence: Synthetic oligonucleotide"
  source 1..18: mol_type = other DNA
ggtggcggaggaagcggt

SEQ ID NO: 32 - DNA, 21 bp, synthetic construct
  misc_feature 1..21: note = source = /note="Description of Artificial Sequence: Synthetic oligonucleotide"
  source 1..21: mol_type = other DNA
ggtggcggaggaagcggtggc

SEQ ID NO: 33 - DNA, 24 bp, synthetic construct
  misc_feature 1..24: note = source = /note="Description of Artificial Sequence: Synthetic oligonucleotide"
  source 1..24: mol_type = other DNA
ggtggcggaggaagcggtggcggc

SEQ ID NO: 34 - DNA, 27 bp, synthetic construct
  misc_feature 1..27: note = source = /note="Description of Artificial Sequence: Synthetic oligonucleotide"
  source 1..27: mol_type = other DNA
ggtggcggaggaagcggtggcggcgga

SEQ ID NO: 35 - DNA, 30 bp, synthetic construct
  misc_feature 1..30: note = source = /note="Description of Artificial Sequence: Synthetic oligonucleotide"
  source 1..30: mol_type = other DNA
ggtggcggaggaagcggtggcggcggatct

SEQ ID NO: 36 - DNA, 360 bp, synthetic construct
  misc_feature 1..360: note = source = /note="Description of Artificial Sequence: Synthetic polynucleotide"
  source 1..360: mol_type = other DNA
accatcaagccttgtcctccatgcaagtgccccgctcctaatctgctcggaggcccttccgtgttcatcttcccacctaagatcaaggacgtgctgatgatctccctgtctcctatcgtgacctgcgtggtggtggacgtgtccgaggatgatcctgacgtgcagatcagttggttcgtgaacaacgtggaagtgcacaccgctcagacccagacacacagagaggactacaacagcaccctgagagtggtgtctgccctgcctatccagcaccaggattggatgtccggcaaagaattcaagtgcaaagtgaacaacaaggacctgcctgctccaatcgagcggaccatctccaagcct

SEQ ID NO: 37 - DNA, 348 bp, synthetic construct
  misc_feature 1..348: note = source = /note="Description of Artificial Sequence: Synthetic polynucleotide"
  source 1..348: mol_type = other DNA
aagcctaacatccagaatcctgagcctgccgtgtaccagctgaaggaccctagatctcaggactctaccctgtgcctgttcaccgacttcgactcccagatcaacgtgcccaagaccatggaatccggcaccttcatcaccgataagtgcgtgctggacatgaaggccatggactccaagtccaacggcgctatcgcctggtccaaccagaccagcttcacatgccaggacatcttcaaagagacaaacgccacctatccttccagcgacgtgccctgtgatgctaccctgaccgagaagtccttcgagacagacatgaacctgaacttccagaacctgtcctgatga

SEQ ID NO: 38 - DNA, 390 bp, synthetic construct
  misc_feature 1..390: note = source = /note="Description of Artificial Sequence: Synthetic polynucleotide"
  source 1..390: mol_type = other DNA
gtggtggaagatctgcggaacgtgacccctcctaaggtgtccctgttcgagccttccaaggccgagatcgccaacaagcagaaagctaccctcgtgtgcctggccagaggcttctttcctgaccacgtggaactgtcttggtgggtcaacggcaaagaggtgcactccggcgtctgtaccgatcctcaggcctacaaagagtccaactactcctacagcctgtcctctcggctgagagtgtctgccaccttctggcacaaccctcggaaccacttcagatgccaggtgcagtttcacggcctgtccgaagaggacaagtggcctgagggatcccctaagcctgtgacacagaacatctctgccgaggcctggggtagagctgatggtggc

SEQ ID NO: 39 - DNA, 372 bp, synthetic construct
  misc_feature 1..372: note = source = /note="Description of Artificial Sequence: Synthetic polynucleotide"
  source 1..372: mol_type = other DNA
ctggaacagctgctgatggacctgcaagagctgctgtcccggatggaaaactaccggaacctgaagctgccccggatgctgaccgctaagttcgctctgcctaagcaggccaccgagctgaaggatctgcagtgcctggaagatgagctgggccctctgagacacgtgctggatctgacccagtccaagtcctttcagctcgaggacgccgagaacttcatctccaacatcagagtgaccgtggtcaagctgaagggctccgacaacaccttcgagtgccagttcgacgatgagtccgctacagtggtggacttcctgcggagatggatcgccttctgccagtccatcatctccacctctccacagtgatga

SEQ ID NO: 40 - DNA, 45 bp, synthetic construct
  misc_feature 1..45: note = source = /note="Description of Artificial Sequence: Synthetic oligonucleotide"
  source 1..45: mol_type = other DNA
ggaggatctggcggaggtggaagcggcggaggcggatcttctcat

SEQ ID NO: 41 - DNA, 321 bp, synthetic construct
  misc_feature 1..321: note = source = /note="Description of Artificial Sequence: Synthetic polynucleotide"
  source 1..321: mol_type = other DNA
ggccagcctagggaaccccaggtttacaccctgcctccatgccgggaagagatgaccaagaaccaggtgtccctgtggtgcctggttaagggcttctacccctccgatatcgccgtggaatgggagtctaatggccagcctgagaacaactacaagacaacccctcctgtgctggactccgacggctcattcttcctgtactccaagctgacagtggacaagtccagatggcagcagggcaacgtgttctcctgctccgtgatgcacgaggccctgcacaatcactacacccagaagtccctgtctctgagccccggcaag

SEQ ID NO: 42 - DNA, 320 bp, synthetic construct
  misc_feature 1..320: note = source = /note="Description of Artificial Sequence: Synthetic polynucleotide"
  source 1..320: mol_type = other DNA
gccagcctcgggaacctcaagtctgtaccctgcctcctagccgggaagagatgaccaagaaccaggtgtccctgtcctgcgctgtgaagggcttctacccttccgatatcgccgtggaatgggagagcaatggccagcctgagaacaactacaagaccacacctcctgtgctggactccgacggctcattcttcctggtgtccaagctgacagtggacaagtccagatggcagcagggcaacgtgttctcctgctccgtgatgcacgaggccctgcacaatcactacacccagaagtccctgtctctgagccccggcaag

SEQ ID NO: 43 - DNA, 1302 bp, synthetic construct
  misc_feature 1..1302: note = source = /note="Description of Artificial Sequence: Synthetic polynucleotide"
  source 1..1302: mol_type = other DNA
caggtgcagctggtggaatctggtggcggagttgtgcagcctggcagatccctgagactgtcttgtgccgcctccggcttcaccttctccagctacaccatgcactgggtccgacaggcccctggcaaaggattggagtgggtcaccttcatctcttacgacggcaacaacaagtactacgccgactccgtgaagggcagattcaccatctctcgggacaactccaagaacaccctgtacctgcagatgaactccctgagagccgaggacaccgccatctactactgtgctagaaccggctggctgggcccctttgattattggggacagggcaccctggtcaccgtgtcctctgcttccaccaagggaccctctgtgttccctctggctccttccagcaagtctacctctggcggaacagctgctctgggctgcctggtcaaggactactttcctgagcctgtgaccgtgtcttggaactctggcgctctgacatccggcgtgcacacctttccagctgtgctgcaatcctccggcctgtactctctgtcctccgtcgtgaccgtgccttctagctctctgggcacccagacctacatctgcaatgtgaaccacaagccttccaacaccaaggtggacaagagagtggaacccaagtcctgcgataagacccacacctgtccaccatgtcctgctccagaactgctcggcggaccttccgtgttcctgtttcctccaaagcctaaggacaccctgatgatctctcggacccctgaagtgacctgcgtggtggtggatgtgtctcacgaggatcccgaagtgaagttcaattggtacgtggacggcgtggaagtgcacaacgccaagaccaagcctagagaggaacagtacaactccacctacagagtggtgtccgtgctgaccgtgctgcaccaggattggctgaacggcaaagagtacaagtgcaaggtgtccaacaaggccctgcctgctcctatcgaaaagaccatctccaaggccaaacctgacattcagaaccccgatcctgccgtgtaccagctgagagactccaagtcctccgataagtctgtgtgcctgttcaccgacttcgactcccagaccaacgtgtcccagtccaaggactccgacgtgtacatcaccgataagtgcgtgctggacatgcggagcatggacttcaagtctaactccgccgtggcctggtctaacaagtccgatttcgcctgcgccaacgccttcaacaacagcattatccccgaggacacattcttcccatcacctgag

SEQ ID NO: 44 - DNA, 1305 bp, synthetic construct
  misc_feature 1..1305: note = source = /note="Description of Artificial Sequence: Synthetic polynucleotide"
  source 1..1305: mol_type = other DNA
caggtgcagctggtggaatctggtggcggagttgtgcagcctggcagatccctgagactgtcttgtgccgcctccggcttcaccttctccagctacaccatgcactgggtccgacaggcccctggcaaaggattggagtgggtcaccttcatctcttacgacggcaacaacaagtactacgccgactccgtgaagggcagattcaccatctctcgggacaactccaagaacaccctgtacctgcagatgaactccctgagagccgaggacaccgccatctactactgtgctagaaccggctggctgggcccctttgattattggggacagggcaccctggtcaccgtgtcctctgcttccaccaagggaccctctgtgttccctctggctccttccagcaagtctacctctggcggaacagctgctctgggctgcctggtcaaggactactttcctgagcctgtgaccgtgtcttggaactctggcgctctgacatccggcgtgcacacctttccagctgtgctgcaatcctccggcctgtactctctgtcctccgtcgtgaccgtgccttctagctctctgggcacccagacctacatctgcaatgtgaaccacaagccttccaacaccaaggtggacaagagagtggaacccaagtcctgcgataagacccacacctgtccaccatgtcctgctccagaactgctcggcggaccttccgtgttcctgtttcctccaaagcctaaggacaccctgatgatctctcggacccctgaagtgacctgcgtggtggtggatgtgtctcacgaggatcccgaagtgaagttcaattggtacgtggacggcgtggaagtgcacaacgccaagaccaagcctagagaggaacagtacaactccacctacagagtggtgtccgtgctgaccgtgctgcaccaggattggctgaacggcaaagagtacaagtgcaaggtgtccaacaaggccctgcctgctcctatcgaaaagaccatctccaaggccaaaggtcctgacattcagaaccccgatcctgccgtgtaccagctgagagactccaagtcctccgataagtctgtgtgcctgttcaccgacttcgactcccagaccaacgtgtcccagtccaaggactccgacgtgtacatcaccgataagtgcgtgctggacatgcggagcatggacttcaagtctaactccgccgtggcctggtctaacaagtccgatttcgcctgcgccaacgccttcaacaacagcattatccccgaggacacattcttcccatcacctgag

SEQ ID NO: 45 - DNA, 1308 bp, synthetic construct
  misc_feature 1..1308: note = source = /note="Description of Artificial Sequence: Synthetic polynucleotide"
  source 1..1308: mol_type = other DNA
caggtgcagctggtggaatctggtggcggagttgtgcagcctggcagatccctgagactgtcttgtgccgcctccggcttcaccttctccagctacaccatgcactgggtccgacaggcccctggcaaaggattggagtgggtcaccttcatctcttacgacggcaacaacaagtactacgccgactccgtgaagggcagattcaccatctctcgggacaactccaagaacaccctgtacctgcagatgaactccctgagagccgaggacaccgccatctactactgtgctagaaccggctggctgggcccctttgattattggggacagggcaccctggtcaccgtgtcctctgcttccaccaagggaccctctgtgttccctctggctccttccagcaagtctacctctggcggaacagctgctctgggctgcctggtcaaggactactttcctgagcctgtgaccgtgtcttggaactctggcgctctgacatccggcgtgcacacctttccagctgtgctgcaatcctccggcctgtactctctgtcctccgtcgtgaccgtgccttctagctctctgggcacccagacctacatctgcaatgtgaaccacaagccttccaacaccaaggtggacaagagagtggaacccaagtcctgcgataagacccacacctgtccaccatgtcctgctccagaactgctcggcggaccttccgtgttcctgtttcctccaaagcctaaggacaccctgatgatctctcggacccctgaagtgacctgcgtggtggtggatgtgtctcacgaggatcccgaagtgaagttcaattggtacgtggacggcgtggaagtgcacaacgccaagaccaagcctagagaggaacagtacaactccacctacagagtggtgtccgtgctgaccgtgctgcaccaggattggctgaacggcaaagagtacaagtgcaaggtgtccaacaaggccctgcctgctcctatcgaaaagaccatctccaaggccaaaggtggccctgacattcagaaccccgatcctgccgtgtaccagctgagagactccaagtcctccgataagtctgtgtgcctgttcaccgacttcgactcccagaccaacgtgtcccagtccaaggactccgacgtgtacatcaccgataagtgcgtgctggacatgcggagcatggacttcaagtctaactccgccgtggcctggtctaacaagtccgatttcgcctgcgccaacgccttcaacaacagcattatccccgaggacacattcttcccatcacctgag

SEQ ID NO: 46 - DNA, 1311 bp, synthetic construct
  misc_feature 1..1311: note = source = /note="Description of Artificial Sequence: Synthetic polynucleotide"
  source 1..1311: mol_type = other DNA
caggtgcagctggtggaatctggtggcggagttgtgcagcctggcagatccctgagactgtcttgtgccgcctccggcttcaccttctccagctacaccatgcactgggtccgacaggcccctggcaaaggattggagtgggtcaccttcatctcttacgacggcaacaacaagtactacgccgactccgtgaagggcagattcaccatctctcgggacaactccaagaacaccctgtacctgcagatgaactccctgagagccgaggacaccgccatctactactgtgctagaaccggctggctgggcccctttgattattggggacagggcaccctggtcaccgtgtcctctgcttccaccaagggaccctctgtgttccctctggctccttccagcaagtctacctctggcggaacagctgctctgggctgcctggtcaaggactactttcctgagcctgtgaccgtgtcttggaactctggcgctctgacatccggcgtgcacacctttccagctgtgctgcaatcctccggcctgtactctctgtcctccgtcgtgaccgtgccttctagctctctgggcacccagacctacatctgcaatgtgaaccacaagccttccaacaccaaggtggacaagagagtggaacccaagtcctgcgataagacccacacctgtccaccatgtcctgctccagaactgctcggcggaccttccgtgttcctgtttcctccaaagcctaaggacaccctgatgatctctcggacccctgaagtgacctgcgtggtggtggatgtgtctcacgaggatcccgaagtgaagttcaattggtacgtggacggcgtggaagtgcacaacgccaagaccaagcctagagaggaacagtacaactccacctacagagtggtgtccgtgctgaccgtgctgcaccaggattggctgaacggcaaagagtacaagtgcaaggtgtccaacaaggccctgcctgctcctatcgaaaagaccatctccaaggccaaaggtggcggacctgacattcagaaccccgatcctgccgtgtaccagctgagagactccaagtcctccgataagtctgtgtgcctgttcaccgacttcgactcccagaccaacgtgtcccagtccaaggactccgacgtgtacatcaccgataagtgcgtgctggacatgcggagcatggacttcaagtctaactccgccgtggcctggtctaacaagtccgatttcgcctgcgccaacgccttcaacaacagcattatccccgaggacacattcttcccatcacctgag

SEQ ID NO: 47 - DNA, 1314 bp, synthetic construct
  misc_feature 1..1314: note = source = /note="Description of Artificial Sequence: Synthetic polynucleotide"
  source 1..1314: mol_type = other DNA
caggtgcagctggtggaatctggtggcggagttgtgcagcctggcagatccctgagactgtcttgtgccgcctccggcttcaccttctccagctacaccatgcactgggtccgacaggcccctggcaaaggattggagtgggtcaccttcatctcttacgacggcaacaacaagtactacgccgactccgtgaagggcagattcaccatctctcgggacaactccaagaacaccctgtacctgcagatgaactccctgagagccgaggacaccgccatctactactgtgctagaaccggctggctgggcccctttgattattggggacagggcaccctggtcaccgtgtcctctgcttccaccaagggaccctctgtgttccctctggctccttccagcaagtctacctctggcggaacagctgctctgggctgcctggtcaaggactactttcctgagcctgtgaccgtgtcttggaactctggcgctctgacatccggcgtgcacacctttccagctgtgctgcaatcctccggcctgtactctctgtcctccgtcgtgaccgtgccttctagctctctgggcacccagacctacatctgcaatgtgaaccacaagccttccaacaccaaggtggacaagagagtggaacccaagtcctgcgataagacccacacctgtccaccatgtcctgctccagaactgctcggcggaccttccgtgttcctgtttcctccaaagcctaaggacaccctgatgatctctcggacccctgaagtgacctgcgtggtggtggatgtgtctcacgaggatcccgaagtgaagttcaattggtacgtggacggcgtggaagtgcacaacgccaagaccaagcctagagaggaacagtacaactccacctacagagtggtgtccgtgctgaccgtgctgcaccaggattggctgaacggcaaagagtacaagtgcaaggtgtccaacaaggccctgcctgctcctatcgaaaagaccatctccaaggccaaaggtggcggaggacctgacattcagaaccccgatcctgccgtgtaccagctgagagactccaagtcctccgataagtctgtgtgcctgttcaccgacttcgactcccagaccaacgtgtcccagtccaaggactccgacgtgtacatcaccgataagtgcgtgctggacatgcggagcatggacttcaagtctaactccgccgtggcctggtctaacaagtccgatttcgcctgcgccaacgccttcaacaacagcattatccccgaggacacattcttcccatcacctgag

SEQ ID NO: 48 - DNA, 1317 bp, synthetic construct
  misc_feature 1..1317: note = source = /note="Description of Artificial Sequence: Synthetic polynucleotide"
  source 1..1317: mol_type = other DNA
caggtgcagctggtggaatctggtggcggagttgtgcagcctggcagatccctgagactgtcttgtgccgcctccggcttcaccttctccagctacaccatgcactgggtccgacaggcccctggcaaaggattggagtgggtcaccttcatctcttacgacggcaacaacaagtactacgccgactccgtgaagggcagattcaccatctctcgggacaactccaagaacaccctgtacctgcagatgaactccctgagagccgaggacaccgccatctactactgtgctagaaccggctggctgggcccctttgattattggggacagggcaccctggtcaccgtgtcctctgcttccaccaagggaccctctgtgttccctctggctccttccagcaagtctacctctggcggaacagctgctctgggctgcctggtcaaggactactttcctgagcctgtgaccgtgtcttggaactctggcgctctgacatccggcgtgcacacctttccagctgtgctgcaatcctccggcctgtactctctgtcctccgtcgtgaccgtgccttctagctctctgggcacccagacctacatctgcaatgtgaaccacaagccttccaacaccaaggtggacaagagagtggaacccaagtcctgcgataagacccacacctgtccaccatgtcctgctccagaactgctcggcggaccttccgtgttcctgtttcctccaaagcctaaggacaccctgatgatctctcggacccctgaagtgacctgcgtggtggtggatgtgtctcacgaggatcccgaagtgaagttcaattggtacgtggacggcgtggaagtgcacaacgccaagaccaagcctagagaggaacagtacaactccacctacagagtggtgtccgtgctgaccgtgctgcaccaggattggctgaacggcaaagagtacaagtgcaaggtgtccaacaaggccctgcctgctcctatcgaaaagaccatctccaaggccaaaggtggcggaggaagccctgacattcagaaccccgatcctgccgtgtaccagctgagagactccaagtcctccgataagtctgtgtgcctgttcaccgacttcgactcccagaccaacgtgtcccagtccaaggactccgacgtgtacatcaccgataagtgcgtgctggacatgcggagcatggacttcaagtctaactccgccgtggcctggtctaacaagtccgatttcgcctgcgccaacgccttcaacaacagcattatccccgaggacacattcttcccatcacctgag

SEQ ID NO: 49 - DNA, 1320 bp, synthetic construct
  misc_feature 1..1320: note = source = /note="Description of Artificial Sequence: Synthetic polynucleotide"
  source 1..1320: mol_type = other DNA
caggtgcagctggtggaatctggtggcggagttgtgcagcctggcagatccctgagactgtcttgtgccgcctccggcttcaccttctccagctacaccatgcactgggtccgacaggcccctggcaaaggattggagtgggtcaccttcatctcttacgacggcaacaacaagtactacgccgactccgtgaagggcagattcaccatctctcgggacaactccaagaacaccctgtacctgcagatgaactccctgagagccgaggacaccgccatctactactgtgctagaaccggctggctgggcccctttgattattggggacagggcaccctggtcaccgtgtcctctgcttccaccaagggaccctctgtgttccctctggctccttccagcaagtctacctctggcggaacagctgctctgggctgcctggtcaaggactactttcctgagcctgtgaccgtgtcttggaactctggcgctctgacatccggcgtgcacacctttccagctgtgctgcaatcctccggcctgtactctctgtcctccgtcgtgaccgtgccttctagctctctgggcacccagacctacatctgcaatgtgaaccacaagccttccaacaccaaggtggacaagagagtggaacccaagtcctgcgataagacccacacctgtccaccatgtcctgctccagaactgctcggcggaccttccgtgttcctgtttcctccaaagcctaaggacaccctgatgatctctcggacccctgaagtgacctgcgtggtggtggatgtgtctcacgaggatcccgaagtgaagttcaattggtacgtggacggcgtggaagtgcacaacgccaagaccaagcctagagaggaacagtacaactccacctacagagtggtgtccgtgctgaccgtgctgcaccaggattggctgaacggcaaagagtacaagtgcaaggtgtccaacaaggccctgcctgctcctatcgaaaagaccatctccaaggccaaaggtggcggaggaagcggtcctgacattcagaaccccgatcctgccgtgtaccagctgagagactccaagtcctccgataagtctgtgtgcctgttcaccgacttcgactcccagaccaacgtgtcccagtccaaggactccgacgtgtacatcaccgataagtgcgtgctggacatgcggagcatggacttcaagtctaactccgccgtggcctggtctaacaagtccgatttcgcctgcgccaacgccttcaacaacagcattatccccgaggacacattcttcccatcacctgag

SEQ ID NO: 50 - DNA, 1323 bp, synthetic construct
  misc_feature 1..1323: note = source = /note="Description of Artificial Sequence: Synthetic polynucleotide"
  source 1..1323: mol_type = other DNA
caggtgcagctggtggaatctggtggcggagttgtgcagcctggcagatccctgagactgtcttgtgccgcctccggcttcaccttctccagctacaccatgcactgggtccgacaggcccctggcaaaggattggagtgggtcaccttcatctcttacgacggcaacaacaagtactacgccgactccgtgaagggcagattcaccatctctcgggacaactccaagaacaccctgtacctgcagatgaactccctgagagccgaggacaccgccatctactactgtgctagaaccggctggctgggcccctttgattattggggacagggcaccctggtcaccgtgtcctctgcttccaccaagggaccctctgtgttccctctggctccttccagcaagtctacctctggcggaacagctgctctgggctgcctggtcaaggactactttcctgagcctgtgaccgtgtcttggaactctggcgctctgacatccggcgtgcacacctttccagctgtgctgcaatcctccggcctgtactctctgtcctccgtcgtgaccgtgccttctagctctctgggcacccagacctacatctgcaatgtgaaccacaagccttccaacaccaaggtggacaagagagtggaacccaagtcctgcgataagacccacacctgtccaccatgtcctgctccagaactgctcggcggaccttccgtgttcctgtttcctccaaagcctaaggacaccctgatgatctctcggacccctgaagtgacctgcgtggtggtggatgtgtctcacgaggatcccgaagtgaagttcaattggtacgtggacggcgtggaagtgcacaacgccaagaccaagcctagagaggaacagtacaactccacctacagagtggtgtccgtgctgaccgtgctgcaccaggattggctgaacggcaaagagtacaagtgcaaggtgtccaacaaggccctgcctgctcctatcgaaaagaccatctccaaggccaaaggtggcggaggaagcggtggccctgacattcagaaccccgatcctgccgtgtaccagctgagagactccaagtcctccgataagtctgtgtgcctgttcaccgacttcgactcccagaccaacgtgtcccagtccaaggactccgacgtgtacatcaccgataagtgcgtgctggacatgcggagcatggacttcaagtctaactccgccgtggcctggtctaacaagtccgatttcgcctgcgccaacgccttcaacaacagcattatccccgaggacacattcttcccatcacctgag

SEQ ID NO: 51 - DNA, 1326 bp, synthetic construct
  misc_feature 1..1326: note = source = /note="Description of Artificial Sequence: Synthetic polynucleotide"
  source 1..1326: mol_type = other DNA
caggtgcagctggtggaatctggtggcggagttgtgcagcctggcagatccctgagactgtcttgtgccgcctccggcttcaccttctccagctacaccatgcactgggtccgacaggcccctggcaaaggattggagtgggtcaccttcatctcttacgacggcaacaacaagtactacgccgactccgtgaagggcagattcaccatctctcgggacaactccaagaacaccctgtacctgcagatgaactccctgagagccgaggacaccgccatctactactgtgctagaaccggctggctgggcccctttgattattggggacagggcaccctggtcaccgtgtcctctgcttccaccaagggaccctctgtgttccctctggctccttccagcaagtctacctctggcggaacagctgctctgggctgcctggtcaaggactactttcctgagcctgtgaccgtgtcttggaactctggcgctctgacatccggcgtgcacacctttccagctgtgctgcaatcctccggcctgtactctctgtcctccgtcgtgaccgtgccttctagctctctgggcacccagacctacatctgcaatgtgaaccacaagccttccaacaccaaggtggacaagagagtggaacccaagtcctgcgataagacccacacctgtccaccatgtcctgctccagaactgctcggcggaccttccgtgttcctgtttcctccaaagcctaaggacaccctgatgatctctcggacccctgaagtgacctgcgtggtggtggatgtgtctcacgaggatcccgaagtgaagttcaattggtacgtggacggcgtggaagtgcacaacgccaagaccaagcctagagaggaacagtacaactccacctacagagtggtgtccgtgctgaccgtgctgcaccaggattggctgaacggcaaagagtacaagtgcaaggtgtccaacaaggccctgcctgctcctatcgaaaagaccatctccaaggccaaaggtggcggaggaagcggtggcggccctgacattcagaaccccgatcctgccgtgtaccagctgagagactccaagtcctccgataagtctgtgtgcctgttcaccgacttcgactcccagaccaacgtgtcccagtccaaggactccgacgtgtacatcaccgataagtgcgtgctggacatgcggagcatggacttcaagtctaactccgccgtggcctggtctaacaagtccgatttcgcctgcgccaacgccttcaacaacagcattatccccgaggacacattcttcccatcacctgag

SEQ ID NO: 52 - DNA, 1329 bp, synthetic construct
  misc_feature 1..1329: note = source = /note="Description of Artificial Sequence: Synthetic polynucleotide"
  source 1..1329: mol_type = other DNA
caggtgcagctggtggaatctggtggcggagttgtgcagcctggcagatccctgagactgtcttgtgccgcctccggcttcaccttctccagctacaccatgcactgggtccgacaggcccctggcaaaggattggagtgggtcaccttcatctcttacgacggcaacaacaagtactacgccgactccgtgaagggcagattcaccatctctcgggacaactccaagaacaccctgtacctgcagatgaactccctgagagccgaggacaccgccatctactactgtgctagaaccggctggctgggcccctttgattattggggacagggcaccctggtcaccgtgtcctctgcttccaccaagggaccctctgtgttccctctggctccttccagcaagtctacctctggcggaacagctgctctgggctgcctggtcaaggactactttcctgagcctgtgaccgtgtcttggaactctggcgctctgacatccggcgtgcacacctttccagctgtgctgcaatcctccggcctgtactctctgtcctccgtcgtgaccgtgccttctagctctctgggcacccagacctacatctgcaatgtgaaccacaagccttccaacaccaaggtggacaagagagtggaacccaagtcctgcgataagacccacacctgtccaccatgtcctgctccagaactgctcggcggaccttccgtgttcctgtttcctccaaagcctaaggacaccctgatgatctctcggacccctgaagtgacctgcgtggtggtggatgtgtctcacgaggatcccgaagtgaagttcaattggtacgtggacggcgtggaagtgcacaacgccaagaccaagcctagagaggaacagtacaactccacctacagagtggtgtccgtgctgaccgtgctgcaccaggattggctgaacggcaaagagtacaagtgcaaggtgtccaacaaggccctgcctgctcctatcgaaaagaccatctccaaggccaaaggtggcggaggaagcggtggcggcggacctgacattcagaaccccgatcctgccgtgtaccagctgagagactccaagtcctccgataagtctgtgtgcctgttcaccgacttcgactcccagaccaacgtgtcccagtccaaggactccgacgtgtacatcaccgataagtgcgtgctggacatgcggagcatggacttcaagtctaactccgccgtggcctggtctaacaagtccgatttcgcctgcgccaacgccttcaacaacagcattatccccgaggacacattcttcccatcacctgag

SEQ ID NO: 53 - DNA, 1332 bp, synthetic construct
  misc_feature 1..1332: note = source = /note="Description of Artificial Sequence: Synthetic polynucleotide"
  source 1..1332: mol_type = other DNA
caggtgcagctggtggaatctggtggcggagttgtgcagcctggcagatccctgagactgtcttgtgccgcctccggcttcaccttctccagctacaccatgcactgggtccgacaggcccctggcaaaggattggagtgggtcaccttcatctcttacgacggcaacaacaagtactacgccgactccgtgaagggcagattcaccatctctcgggacaactccaagaacaccctgtacctgcagatgaactccctgagagccgaggacaccgccatctactactgtgctagaaccggctggctgggcccctttgattattggggacagggcaccctggtcaccgtgtcctctgcttccaccaagggaccctctgtgttccctctggctccttccagcaagtctacctctggcggaacagctgctctgggctgcctggtcaaggactactttcctgagcctgtgaccgtgtcttggaactctggcgctctgacatccggcgtgcacacctttccagctgtgctgcaatcctccggcctgtactctctgtcctccgtcgtgaccgtgccttctagctctctgggcacccagacctacatctgcaatgtgaaccacaagccttccaacaccaaggtggacaagagagtggaacccaagtcctgcgataagacccacacctgtccaccatgtcctgctccagaactgctcggcggaccttccgtgttcctgtttcctccaaagcctaaggacaccctgatgatctctcggacccctgaagtgacctgcgtggtggtggatgtgtctcacgaggatcccgaagtgaagttcaattggtacgtggacggcgtggaagtgcacaacgccaagaccaagcctagagaggaacagtacaactccacctacagagtggtgtccgtgctgaccgtgctgcaccaggattggctgaacggcaaagagtacaagtgcaaggtgtccaacaaggccctgcctgctcctatcgaaaagaccatctccaaggccaaaggtggcggaggaagcggtggcggcggatctcctgacattcagaaccccgatcctgccgtgtaccagctgagagactccaagtcctccgataagtctgtgtgcctgttcaccgacttcgactcccagaccaacgtgtcccagtccaaggactccgacgtgtacatcaccgataagtgcgtgctggacatgcggagcatggacttcaagtctaactccgccgtggcctggtctaacaagtccgatttcgcctgcgccaacgccttcaacaacagcattatccccgaggacacattcttcccatcacctgag

SEQ ID NO: 54 - DNA, 645 bp, synthetic construct
  misc_feature 1..645: note = source = /note="Description of Artificial Sequence: Synthetic polynucleotide"
  source 1..645: mol_type = other DNA
gagatcgtgctgacccagtctcctggcacactgtcactgtctccaggcgagagagctaccctgtcctgtagagcctctcagtccgtgggctcctcttacctggcttggtatcagcagaagcccggccaggctcctagactgttgatctacggcgccttctccagagccacaggcatccctgatagattctccggctctggctctggcaccgacttcaccctgaccatctccagactggaacccgaggacttcgccgtgtactactgtcagcagtacggctcctctccttggacctttggccagggcaccaaggtggaaatcaagcggacagtggccgctccttccgtgttcatcttcccaccttccgacgagcagctgaagtccggcacagcttctgtcgtgtgcctgctgaacaacttctaccctcgggaagccaaggtgcagtggaaggtggacaatgccctgcagtccggcaactcccaagagtctgtgaccgagcaggactccaaggacagcacctacagcctgtcctccacactgaccctgtccaaggccgactacgagaagcacaaggtgtacgcctgcgaagtgacccatcagggcctgtctagccctgtgaccaagtctttcaaccggggcgagtgc

SEQ ID NO: 55 - DNA, 1404 bp, synthetic construct
  misc_feature 1..1404: note = source = /note="Description of Artificial Sequence: Synthetic polynucleotide"
  source 1..1404: mol_type = other DNA
caggtgcagctggtggaatctggtggcggagttgtgcagcctggcagatccctgagactgtcttgtgccgcctccggcttcaccttctcctcttacggaatgcactgggtccgacaggcccctggcaaaggattggagtgggtcgccttcatcagatacgacggctccaacaagtactacgccgactccgtgaagggcagattcaccatctctcgggacaactccaagaacaccctgtacctgcagatgaactccctgagagccgaggacaccgccgtgtactactgcaagacccacggctctcacgacaattggggccagggcacaatggtcaccgtgtcctctgcttccaccaagggaccctctgtgttccctctggctccttccagcaagtctacctctggcggaacagctgctctgggctgcctggtcaaggactactttcctgagcctgtgaccgtgtcttggaactctggcgctctgacatccggcgtgcacacctttccagctgtgctgcaatcctccggcctgtactctctgtcctccgtcgtgaccgtgccttctagctctctgggcacccagacctacatctgcaatgtgaaccacaagccttccaacaccaaggtggacaagagagtggaacccaagtcctgcgataagacccacacctgtccaccatgtcctgctccagaactgctcggcggaccttccgtgttcctgtttcctccaaagcctaaggacaccctgatgatctctcggacccctgaagtgacctgcgtggtggtggatgtgtctcacgaggatcccgaagtgaagttcaattggtacgtggacggcgtggaagtgcacaacgccaagaccaagcctagagaggaacagtacaactccacctacagagtggtgtccgtgctgaccgtgctgcaccaggattggctgaacggcaaagagtacaagtgcaaggtgtccaacaaggccctgcctgctcctatcgaaaagaccatctccaaggccaaagaggacctgaacaaggttttcccacctgaggtggccctgttcgagccttctgaggctgagatctctcacacccagaaagctaccctcgtgtgtctggccaccggcttctaccctgatcacgtggaactgtcttggtgggtcaacggaaaagaggtgcactccggcgtctgcaccgatcctcagcctctgaaagaacagcccgctctgaacgactccagatacgccctgtcctctcggctgagagtgtctgccaccttctggcaggaccctcggaaccactttagatgccaggtgcagttctacggcctgtccgaggctgatgagtggacccaggctagagccaagccagtgacacagatcgtgtctgccgaagcctggggcagagccgat

SEQ ID NO: 56 - DNA, 1407 bp, synthetic construct
  misc_feature 1..1407: note = source = /note="Description of Artificial Sequence: Synthetic polynucleotide"
  source 1..1407: mol_type = other DNA
caggtgcagctggtggaatctggtggcggagttgtgcagcctggcagatccctgagactgtcttgtgccgcctccggcttcaccttctcctcttacggaatgcactgggtccgacaggcccctggcaaaggattggagtgggtcgccttcatcagatacgacggctccaacaagtactacgccgactccgtgaagggcagattcaccatctctcgggacaactccaagaacaccctgtacctgcagatgaactccctgagagccgaggacaccgccgtgtactactgcaagacccacggctctcacgacaattggggccagggcacaatggtcaccgtgtcctctgcttccaccaagggaccctctgtgttccctctggctccttccagcaagtctacctctggcggaacagctgctctgggctgcctggtcaaggactactttcctgagcctgtgaccgtgtcttggaactctggcgctctgacatccggcgtgcacacctttccagctgtgctgcaatcctccggcctgtactctctgtcctccgtcgtgaccgtgccttctagctctctgggcacccagacctacatctgcaatgtgaaccacaagccttccaacaccaaggtggacaagagagtggaacccaagtcctgcgataagacccacacctgtccaccatgtcctgctccagaactgctcggcggaccttccgtgttcctgtttcctccaaagcctaaggacaccctgatgatctctcggacccctgaagtgacctgcgtggtggtggatgtgtctcacgaggatcccgaagtgaagttcaattggtacgtggacggcgtggaagtgcacaacgccaagaccaagcctagagaggaacagtacaactccacctacagagtggtgtccgtgctgaccgtgctgcaccaggattggctgaacggcaaagagtacaagtgcaaggtgtccaacaaggccctgcctgctcctatcgaaaagaccatctccaaggccaaaggtgaggacctgaacaaggttttcccacctgaggtggccctgttcgagccttctgaggctgagatctctcacacccagaaagctaccctcgtgtgtctggccaccggcttctaccctgatcacgtggaactgtcttggtgggtcaacggaaaagaggtgcactccggcgtctgcaccgatcctcagcctctgaaagaacagcccgctctgaacgactccagatacgccctgtcctctcggctgagagtgtctgccaccttctggcaggaccctcggaaccactttagatgccaggtgcagttctacggcctgtccgaggctgatgagtggacccaggctagagccaagccagtgacacagatcgtgtctgccgaagcctggggcagagccgat

SEQ ID NO: 57 - DNA, 1410 bp, synthetic construct
  misc_feature 1..1410: note = source = /note="Description of Artificial Sequence: Synthetic polynucleotide"
  source 1..1410: mol_type = other DNA
caggtgcagctggtggaatctggtggcggagttgtgcagcctggcagatccctgagactgtcttgtgccgcctccggcttcaccttctcctcttacggaatgcactgggtccgacaggcccctggcaaaggattggagtgggtcgccttcatcagatacgacggctccaacaagtactacgccgactccgtgaagggcagattcaccatctctcgggacaactccaagaacaccctgtacctgcagatgaactccctgagagccgaggacaccgccgtgtactactgcaagacccacggctctcacgacaattggggccagggcacaatggtcaccgtgtcctctgcttccaccaagggaccctctgtgttccctctggctccttccagcaagtctacctctggcggaacagctgctctgggctgcctggtcaaggactactttcctgagcctgtgaccgtgtcttggaactctggcgctctgacatccggcgtgcacacctttccagctgtgctgcaatcctccggcctgtactctctgtcctccgtcgtgaccgtgccttctagctctctgggcacccagacctacatctgcaatgtgaaccacaagccttccaacaccaaggtggacaagagagtggaacccaagtcctgcgataagacccacacctgtccaccatgtcctgctccagaactgctcggcggaccttccgtgttcctgtttcctccaaagcctaaggacaccctgatgatctctcggacccctgaagtgacctgcgtggtggtggatgtgtctcacgaggatcccgaagtgaagttcaattggtacgtggacggcgtggaagtgcacaacgccaagaccaagcctagagaggaacagtacaactccacctacagagtggtgtccgtgctgaccgtgctgcaccaggattggctgaacggcaaagagtacaagtgcaaggtgtccaacaaggccctgcctgctcctatcgaaaagaccatctccaaggccaaaggtggcgaggacctgaacaaggttttcccacctgaggtggccctgttcgagccttctgaggctgagatctctcacacccagaaagctaccctcgtgtgtctggccaccggcttctaccctgatcacgtggaactgtcttggtgggtcaacggaaaagaggtgcactccggcgtctgcaccgatcctcagcctctgaaagaacagcccgctctgaacgactccagatacgccctgtcctctcggctgagagtgtctgccaccttctggcaggaccctcggaaccactttagatgccaggtgcagttctacggcctgtccgaggctgatgagtggacccaggctagagccaagccagtgacacagatcgtgtctgccgaagcctggggcagagccgat

SEQ ID NO: 58 - DNA, 1413 bp, synthetic construct
  misc_feature 1..1413: note = source = /note="Description of Artificial Sequence: Synthetic polynucleotide"
  source 1..1413: mol_type = other DNA
caggtgcagctggtggaatctggtggcggagttgtgcagcctggcagatccctgagactgtcttgtgccgcctccggcttcaccttctcctcttacggaatgcactgggtccgacaggcccctggcaaaggattggagtgggtcgccttcatcagatacgacggctccaacaagtactacgccgactccgtgaagggcagattcaccatctctcgggacaactccaagaacaccctgtacctgcagatgaactccctgagagccgaggacaccgccgtgtactactgcaagacccacggctctcacgacaattggggccagggcacaatggtcaccgtgtcctctgcttccaccaagggaccctctgtgttccctctggctccttccagcaagtctacctctggcggaacagctgctctgggctgcctggtcaaggactactttcctgagcctgtgaccgtgtcttggaactctggcgctctgacatccggcgtgcacacctttccagctgtgctgcaatcctccggcctgtactctctgtcctccgtcgtgaccgtgccttctagctctctgggcacccagacctacatctgcaatgtgaaccacaagccttccaacaccaaggtggacaagagagtggaacccaagtcctgcgataagacccacacctgtccaccatgtcctgctccagaactgctcggcggaccttccgtgttcctgtttcctccaaagcctaaggacaccctgatgatctctcggacccctgaagtgacctgcgtggtggtggatgtgtctcacgaggatcccgaagtgaagttcaattggtacgtggacggcgtggaagtgcacaacgccaagaccaagcctagagaggaacagtacaactccacctacagagtggtgtccgtgctgaccgtgctgcaccaggattggctgaacggcaaagagtacaagtgcaaggtgtccaacaaggccctgcctgctcctatcgaaaagaccatctccaaggccaaaggtggcggagaggacctgaacaaggttttcccacctgaggtggccctgttcgagccttctgaggctgagatctctcacacccagaaagctaccctcgtgtgtctggccaccggcttctaccctgatcacgtggaactgtcttggtgggtcaacggaaaagaggtgcactccggcgtctgcaccgatcctcagcctctgaaagaacagcccgctctgaacgactccagatacgccctgtcctctcggctgagagtgtctgccaccttctggcaggaccctcggaaccactttagatgccaggtgcagttctacggcctgtccgaggctgatgagtggacccaggctagagccaagccagtgacacagatcgtgtctgccgaagcctggggcagagccgat

SEQ ID NO: 59 - DNA, 1416 bp, synthetic construct
  misc_feature 1..1416: note = source = /note="Description of Artificial Sequence: Synthetic polynucleotide"
  source 1..1416: mol_type = other DNA
caggtgcagctggtggaatctggtggcggagttgtgcagcctggcagatccctgagactgtcttgtgccgcctccggcttcaccttctcctcttacggaatgcactgggtccgacaggcccctggcaaaggattggagtgggtcgccttcatcagatacgacggctccaacaagtactacgccgactccgtgaagggcagattcaccatctctcgggacaactccaagaacaccctgtacctgcagatgaactccctgagagccgaggacaccgccgtgtactactgcaagacccacggctctcacgacaattggggccagggcacaatggtcaccgtgtcctctgcttccaccaagggaccctctgtgttccctctggctccttccagcaagtctacctctggcggaacagctgctctgggctgcctggtcaaggactactttcctgagcctgtgaccgtgtcttggaactctggcgctctgacatccggcgtgcacacctttccagctgtgctgcaatcctccggcctgtactctctgtcctccgtcgtgaccgtgccttctagctctctgggcacccagacctacatctgcaatgtgaaccacaagccttccaacaccaaggtggacaagagagtggaacccaagtcctgcgataagacccacacctgtccaccatgtcctgctccagaactgctcggcggaccttccgtgttcctgtttcctccaaagcctaaggacaccctgatgatctctcggacccctgaagtgacctgcgtggtggtggatgtgtctcacgaggatcccgaagtgaagttcaattggtacgtggacggcgtggaagtgcacaacgccaagaccaagcctagagaggaacagtacaactccacctacagagtggtgtccgtgctgaccgtgctgcaccaggattggctgaacggcaaagagtacaagtgcaaggtgtccaacaaggccctgcctgctcctatcgaaaagaccatctccaaggccaaaggtggcggaggagaggacctgaacaaggttttcccacctgaggtggccctgttcgagccttctgaggctgagatctctcacacccagaaagctaccctcgtgtgtctggccaccggcttctaccctgatcacgtggaactgtcttggtgggtcaacggaaaagaggtgcactccggcgtctgcaccgatcctcagcctctgaaagaacagcccgctctgaacgactccagatacgccctgtcctctcggctgagagtgtctgccaccttctggcaggaccctcggaaccactttagatgccaggtgcagttctacggcctgtccgaggctgatgagtggacccaggctagagccaagccagtgacacagatcgtgtctgccgaagcctggggcagagccgat

SEQ ID NO: 60 - DNA, 1419 bp, synthetic construct
  misc_feature 1..1419: note = source = /note="Description of Artificial Sequence: Synthetic polynucleotide"
  source 1..1419: mol_type = other DNA
caggtgcagctggtggaatctggtggcggagttgtgcagcctggcagatccctgagactgtcttgtgccgcctccggcttcaccttctcctcttacggaatgcactgggtccgacaggcccctggcaaaggattggagtgggtcgccttcatcagatacgacggctccaacaagtactacgccgactccgtgaagggcagattcaccatctctcgggacaactccaagaacaccctgtacctgcagatgaactccctgagagccgaggacaccgccgtgtactactgcaagacccacggctctcacgacaattggggccagggcacaatggtcaccgtgtcctctgcttccaccaagggaccctctgtgttccctctggctccttccagcaagtctacctctggcggaacagctgctctgggctgcctggtcaaggactactttcctgagcctgtgaccgtgtcttggaactctggcgctctgacatccggcgtgcacacctttccagctgtgctgcaatcctccggcctgtactctctgtcctccgtcgtgaccgtgccttctagctctctgggcacccagacctacatctgcaatgtgaaccacaagccttccaacaccaaggtggacaagagagtggaacccaagtcctgcgataagacccacacctgtccaccatgtcctgctccagaactgctcggcggaccttccgtgttcctgtttcctccaaagcctaaggacaccctgatgatctctcggacccctgaagtgacctgcgtggtggtggatgtgtctcacgaggatcccgaagtgaagttcaattggtacgtggacggcgtggaagtgcacaacgccaagaccaagcctagagaggaacagtacaactccacctacagagtggtgtccgtgctgaccgtgctgcaccaggattggctgaacggcaaagagtacaagtgcaaggtgtccaacaaggccctgcctgctcctatcgaaaagaccatctccaaggccaaaggtggcggaggaagcgaggacctgaacaaggttttcccacctgaggtggccctgttcgagccttctgaggctgagatctctcacacccagaaagctaccctcgtgtgtctggccaccggcttctaccctgatcacgtggaactgtcttggtgggtcaacggaaaagaggtgcactccggcgtctgcaccgatcctcagcctctgaaagaacagcccgctctgaacgactccagatacgccctgtcctctcggctgagagtgtctgccaccttctggcaggaccctcggaaccactttagatgccaggtgcagttctacggcctgtccgaggctgatgagtggacccaggctagagccaagccagtgacacagatcgtgtctgccgaagcctggggcagagccgat

SEQ ID NO: 61 - DNA, 1422 bp, synthetic construct
  misc_feature 1..1422: note = source = /note="Description of Artificial Sequence: Synthetic polynucleotide"
  source 1..1422: mol_type = other DNA
caggtgcagctggtggaatctggtggcggagttgtgcagcctggcagatccctgagactgtcttgtgccgcctccggcttcaccttctcctcttacggaatgcactgggtccgacaggcccctggcaaaggattggagtgggtcgccttcatcagatacgacggctccaacaagtactacgccgactccgtgaagggcagattcaccatctctcgggacaactccaagaacaccctgtacctgcagatgaactccctgagagccgaggacaccgccgtgtactactgcaagacccacggctctcacgacaattggggccagggcacaatggtcaccgtgtcctctgcttccaccaagggaccctctgtgttccctctggctccttccagcaagtctacctctggcggaacagctgctctgggctgcctggtcaaggactactttcctgagcctgtgaccgtgtcttggaactctggcgctctgacatccggcgtgcacacctttccagctgtgctgcaatcctccggcctgtactctctgtcctccgtcgtgaccgtgccttctagctctctgggcacccagacctacatctgcaatgtgaaccacaagccttccaacaccaaggtggacaagagagtggaacccaagtcctgcgataagacccacacctgtccaccatgtcctgctccagaactgctcggcggaccttccgtgttcctgtttcctccaaagcctaaggacaccctgatgatctctcggacccctgaagtgacctgcgtggtggtggatgtgtctcacgaggatcccgaagtgaagttcaattggtacgtggacggcgtggaagtgcacaacgccaagaccaagcctagagaggaacagtacaactccacctacagagtggtgtccgtgctgaccgtgctgcaccaggattggctgaacggcaaagagtacaagtgcaaggtgtccaacaaggccctgcctgctcctatcgaaaagaccatctccaaggccaaaggtggcggaggaagcggtgaggacctgaacaaggttttcccacctgaggtggccctgttcgagccttctgaggctgagatctctcacacccagaaagctaccctcgtgtgtctggccaccggcttctaccctgatcacgtggaactgtcttggtgggtcaacggaaaagaggtgcactccggcgtctgcaccgatcctcagcctctgaaagaacagcccgctctgaacgactccagatacgccctgtcctctcggctgagagtgtctgccaccttctggcaggaccctcggaaccactttagatgccaggtgcagttctacggcctgtccgaggctgatgagtggacccaggctagagccaagccagtgacacagatcgtgtctgccgaagcctggggcagagccgat

SEQ ID NO: 62 - DNA, 1425 bp, synthetic construct
  misc_feature 1..1425: note = source = /note="Description of Artificial Sequence: Synthetic polynucleotide"
  source 1..1425: mol_type = other DNA
caggtgcagctggtggaatctggtggcggagttgtgcagcctggcagatccctgagactgtcttgtgccgcctccggcttcaccttctcctcttacggaatgcactgggtccgacaggcccctggcaaaggattggagtgggtcgccttcatcagatacgacggctccaacaagtactacgccgactccgtgaagggcagattcaccatctctcgggacaactccaagaacaccctgtacctgcagatgaactccctgagagccgaggacaccgccgtgtactactgcaagacccacggctctcacgacaattggggccagggcacaatggtcaccgtgtcctctgcttccaccaagggaccctctgtgttccctctggctccttccagcaagtctacctctggcggaacagctgctctgggctgcctggtcaaggactactttcctgagcctgtgaccgtgtcttggaactctggcgctctgacatccggcgtgcacacctttccagctgtgctgcaatcctccggcctgtactctctgtcctccgtcgtgaccgtgccttctagctctctgggcacccagacctacatctgcaatgtgaaccacaagccttccaacaccaaggtggacaagagagtggaacccaagtcctgcgataagacccacacctgtccaccatgtcctgctccagaactgctcggcggaccttccgtgttcctgtttcctccaaagcctaaggacaccctgatgatctctcggacccctgaagtgacctgcgtggtggtggatgtgtctcacgaggatcccgaagtgaagttcaattggtacgtggacggcgtggaagtgcacaacgccaagaccaagcctagagaggaacagtacaactccacctacagagtggtgtccgtgctgaccgtgctgcaccaggattggctgaacggcaaagagtacaagtgcaaggtgtccaacaaggccctgcctgctcctatcgaaaagaccatctccaaggccaaaggtggcggaggaagcggtggcgaggacctgaacaaggttttcccacctgaggtggccctgttcgagccttctgaggctgagatctctcacacccagaaagctaccctcgtgtgtctggccaccggcttctaccctgatcacgtggaactgtcttggtgggtcaacggaaaagaggtgcactccggcgtctgcaccgatcctcagcctctgaaagaacagcccgctctgaacgactccagatacgccctgtcctctcggctgagagtgtctgccaccttctggcaggaccctcggaaccactttagatgccaggtgcagttctacggcctgtccgaggctgatgagtggacccaggctagagccaagccagtgacacagatcgtgtctgccgaagcctggggcagagccgat

SEQ ID NO: 63 - DNA, 1428 bp, synthetic construct
  misc_feature 1..1428: note = source = /note="Description of Artificial Sequence: Synthetic polynucleotide"
  source 1..1428: mol_type = other DNA
caggtgcagctggtggaatctggtggcggagttgtgcagcctggcagatccctgagactgtcttgtgccgcctccggcttcaccttctcctcttacggaatgcactgggtccgacaggcccctggcaaaggattggagtgggtcgccttcatcagatacgacggctccaacaagtactacgccgactccgtgaagggcagattcaccatctctcgggacaactccaagaacaccctgtacctgcagatgaactccctgagagccgaggacaccgccgtgtactactgcaagacccacggctctcacgacaattggggccagggcacaatggtcaccgtgtcctctgcttccaccaagggaccctctgtgttccctctggctccttccagcaagtctacctctggcggaacagctgctctgggctgcctggtcaaggactactttcctgagcctgtgaccgtgtcttggaactctggcgctctgacatccggcgtgcacacctttccagctgtgctgcaatcctccggcctgtactctctgtcctccgtcgtgaccgtgccttctagctctctgggcacccagacctacatctgcaatgtgaaccacaagccttccaacaccaaggtggacaagagagtggaacccaagtcctgcgataagacccacacctgtccaccatgtcctgctccagaactgctcggcggaccttccgtgttcctgtttcctccaaagcctaaggacaccctgatgatctctcggacccctgaagtgacctgcgtggtggtggatgtgtctcacgaggatcccgaagtgaagttcaattggtacgtggacggcgtggaagtgcacaacgccaagaccaagcctagagaggaacagtacaactccacctacagagtggtgtccgtgctgaccgtgctgcaccaggattggctgaacggcaaagagtacaagtgcaaggtgtccaacaaggccctgcctgctcctatcgaaaagaccatctccaaggccaaaggtggcggaggaagcggtggcggcgaggacctgaacaaggttttcccacctgaggtggccctgttcgagccttctgaggctgagatctctcacacccagaaagctaccctcgtgtgtctggccaccggcttctaccctgatcacgtggaactgtcttggtgggtcaacggaaaagaggtgcactccggcgtctgcaccgatcctcagcctctgaaagaacagcccgctctgaacgactccagatacgccctgtcctctcggctgagagtgtctgccaccttctggcaggaccctcggaaccactttagatgccaggtgcagttctacggcctgtccgaggctgatgagtggacccaggctagagccaagccagtgacacagatcgtgtctgccgaagcctggggcagagccgat

SEQ ID NO: 64 - DNA, 1431 bp, synthetic construct
  misc_feature 1..1431: note = source = /note="Description of Artificial Sequence: Synthetic polynucleotide"
  source 1..1431: mol_type = other DNA
caggtgcagctggtggaatctggtggcggagttgtgcagcctggcagatccctgagactgtcttgtgccgcctccggcttcaccttctcctcttacggaatgcactgggtccgacaggcccctggcaaaggattggagtgggtcgccttcatcagatacgacggctccaacaagtactacgccgactccgtgaagggcagattcaccatctctcgggacaactccaagaacaccctgtacctgcagatgaactccctgagagccgaggacaccgccgtgtactactgcaagacccacggctctcacgacaattggggccagggcacaatggtcaccgtgtcctctgcttccaccaagggaccctctgtgttccctctggctccttccagcaagtctacctctggcggaacagctgctctgggctgcctggtcaaggactactttcctgagcctgtgaccgtgtcttggaactctggcgctctgacatccggcgtgcacacctttccagctgtgctgcaatcctccggcctgtactctctgtcctccgtcgtgaccgtgccttctagctctctgggcacccagacctacatctgcaatgtgaaccacaagccttccaacaccaaggtggacaagagagtggaacccaagtcctgcgataagacccacacctgtccaccatgtcctgctccagaactgctcggcggaccttccgtgttcctgtttcctccaaagcctaaggacaccctgatgatctctcggacccctgaagtgacctgcgtggtggtggatgtgtctcacgaggatcccgaagtgaagttcaattggtacgtggacggcgtggaagtgcacaacgccaagaccaagcctagagaggaacagtacaactccacctacagagtggtgtccgtgctgaccgtgctgcaccaggattggctgaacggcaaagagtacaagtgcaaggtgtccaacaaggccctgcctgctcctatcgaaaagaccatctccaaggccaaaggtggcggaggaagcggtggcggcggagaggacctgaacaaggttttcccacctgaggtggccctgttcgagccttctgaggctgagatctctcacacccagaaagctaccctcgtgtgtctggccaccggcttctaccctgatcacgtggaactgtcttggtgggtcaacggaaaagaggtgcactccggcgtctgcaccgatcctcagcctctgaaagaacagcccgctctgaacgactccagatacgccctgtcctctcggctgagagtgtctgccaccttctggcaggaccctcggaaccactttagatgccaggtgcagttctacggcctgtccgaggctgatgagtggacccaggctagagccaagccagtgacacagatcgtgtctgccgaagcctggggcagagccgat

SEQ ID NO: 65 - DNA, 1434 bp, synthetic construct
  misc_feature 1..1434: note = source = /note="Description of Artificial Sequence: Synthetic polynucleotide"
  source 1..1434: mol_type = other DNA
caggtgcagctggtggaatctggtggcggagttgtgcagcctggcagatccctgagactgtcttgtgccgcctccggcttcaccttctcctcttacggaatgcactgggtccgacaggcccctggcaaaggattggagtgggtcgccttcatcagatacgacggctccaacaagtactacgccgactccgtgaagggcagattcaccatctctcgggacaactccaagaacaccctgtacctgcagatgaactccctgagagccgaggacaccgccgtgtactactgcaagacccacggctctcacgacaattggggccagggcacaatggtcaccgtgtcctctgcttccaccaagggaccctctgtgttccctctggctccttccagcaagtctacctctggcggaacagctgctctgggctgcctggtcaaggactactttcctgagcctgtgaccgtgtcttggaactctggcgctctgacatccggcgtgcacacctttccagctgtgctgcaatcctccggcctgtactctctgtcctccgtcgtgaccgtgccttctagctctctgggcacccagacctacatctgcaatgtgaaccacaagccttccaacaccaaggtggacaagagagtggaacccaagtcctgcgataagacccacacctgtccaccatgtcctgctccagaactgctcggcggaccttccgtgttcctgtttcctccaaagcctaaggacaccctgatgatctctcggacccctgaagtgacctgcgtggtggtggatgtgtctcacgaggatcccgaagtgaagttcaattggtacgtggacggcgtggaagtgcacaacgccaagaccaagcctagagaggaacagtacaactccacctacagagtggtgtccgtgctgaccgtgctgcaccaggattggctgaacggcaaagagtacaagtgcaaggtgtccaacaaggccctgcctgctcctatcgaaaagaccatctccaaggccaaaggtggcggaggaagcggtggcggcggatctgaggacctgaacaaggttttcccacctgaggtggccctgttcgagccttctgaggctgagatctctcacacccagaaagctaccctcgtgtgtctggccaccggcttctaccctgatcacgtggaactgtcttggtgggtcaacggaaaagaggtgcactccggcgtctgcaccgatcctcagcctctgaaagaacagcccgctctgaacgactccagatacgccctgtcctctcggctgagagtgtctgccaccttctggcaggaccctcggaaccactttagatgccaggtgcagttctacggcctgtccgaggctgatgagtggacccaggctagagccaagccagtgacacagatcgtgtctgccgaagcctggggcagagccgat

SEQ ID NO: 66 - DNA, 651 bp, synthetic construct
  misc_feature 1..651: note = source = /note="Description of Artificial Sequence: Synthetic polynucleotide"
  source 1..651: mol_type = other DNA
cagtccgtgttgacccagcctccttctgtttctggcgctcctggccagagagtgaccatctcttgctccggctctcggtccaacatcggctccaataccgtgaagtggtatcagcagctgcccggcacagctcccaaactgctgatctactacaacgaccagcggccttctggcgtgcccgatagattctctggctccaagtctggcacctctgccagcctggctattaccggactgcaggctgaggacgaggccgactactactgccagtcttacgaccggtacacccatcctgctctgctgtttggcaccggcaccaaagtgacagtgctgggccagcctaaggccaatcctaccgtgacactgttccctccatcctccgaagaactgcaggccaacaaggctaccctcgtgtgcctgatctccgacttttaccctggcgctgtgaccgtggcctggaaggctgatggatctcctgtgaaggctggcgtggaaaccaccaagccttccaagcagtccaacaacaaatacgccgcctcctcctacctgtctctgacccctgaacagtggaagtcccaccggtcctacagctgccaagtgacccatgagggctccaccgtggaaaagaccgtggctcctaccgagtgctcc

SEQ ID NO: 67 - DNA, 708 bp, synthetic construct
  misc_feature 1..708: note = source = /note="Description of Artificial Sequence: Synthetic polynucleotide"
  source 1..708: mol_type = other DNA
accatcaagccttgtcctccatgcaagtgccccgctcctaatctgctcggaggcccttccgtgttcatcttcccacctaagatcaaggacgtgctgatgatctccctgtctcctatcgtgacctgcgtggtggtggacgtgtccgaggatgatcctgacgtgcagatcagttggttcgtgaacaacgtggaagtgcacaccgctcagacccagacacacagagaggactacaacagcaccctgagagtggtgtctgccctgcctatccagcaccaggattggatgtccggcaaagaattcaagtgcaaagtgaacaacaaggacctgcctgctccaatcgagcggaccatctccaagcctaagcctaacatccagaatcctgagcctgccgtgtaccagctgaaggaccctagatctcaggactctaccctgtgcctgttcaccgacttcgactcccagatcaacgtgcccaagaccatggaatccggcaccttcatcaccgataagtgcgtgctggacatgaaggccatggactccaagtccaacggcgctatcgcctggtccaaccagaccagcttcacatgccaggacatcttcaaagagacaaacgccacctatccttccagcgacgtgccctgtgatgctaccctgaccgagaagtccttcgagacagacatgaacctgaacttccagaacctgtcctgatga

SEQ ID NO: 68 - DNA, 711 bp, synthetic construct
  misc_feature 1..711: note = source = /note="Description of Artificial Sequence: Synthetic polynucleotide"
  source 1..711: mol_type = other DNA
accatcaagccttgtcctccatgcaagtgccccgctcctaatctgctcggaggcccttccgtgttcatcttcccacctaagatcaaggacgtgctgatgatctccctgtctcctatcgtgacctgcgtggtggtggacgtgtccgaggatgatcctgacgtgcagatcagttggttcgtgaacaacgtggaagtgcacaccgctcagacccagacacacagagaggactacaacagcaccctgagagtggtgtctgccctgcctatccagcaccaggattggatgtccggcaaagaattcaagtgcaaagtgaacaacaaggacctgcctgctccaatcgagcggaccatctccaagcctggtaagcctaacatccagaatcctgagcctgccgtgtaccagctgaaggaccctagatctcaggactctaccctgtgcctgttcaccgacttcgactcccagatcaacgtgcccaagaccatggaatccggcaccttcatcaccgataagtgcgtgctggacatgaaggccatggactccaagtccaacggcgctatcgcctggtccaaccagaccagcttcacatgccaggacatcttcaaagagacaaacgccacctatccttccagcgacgtgccctgtgatgctaccctgaccgagaagtccttcgagacagacatgaacctgaacttccagaacctgtcctgatga

SEQ ID NO: 69 - DNA, 675 bp, synthetic construct
  misc_feature 1..675: note = source = /note="Description of Artificial Sequence: Synthetic polynucleotide"
  source 1..675: mol_type = other DNA
accatcaagccttgtcctccatgcaagtgccccgctcctaatctgctcggaggcccttccgtgttcatcttcccacctaagatcaaggacgtgctgatgatctccctgtctcctatcgtgacctgcgtggtggtggacgtgtccgaggatgatcctgacgtgcagatcagttggttcgtgaacaacgtggaagtgcacaccgctcagacccagacacacagagaggactacaacagcaccctgagagtggtgtctgccctgcctatccagcaccaggattggatgtccggcaaagaattcaagtgcaaagtgaacaacaaggacctgcctgctccaatcgagcggaccatctccaagcctggtggcgcttccaccaagggaccctctgtgttccctctggctccttccagcaagtctacctctggcggaacagctgctctgggctgcctggtcaaggactactttcctgagcctgtgaccgtgtcttggaactctggcgctctgacatccggcgtgcacacctttccagctgtgctgcaatcctccggcctgtactctctgtcctccgtcgtgaccgtgccttctagctctctgggcacccagacctacatctgcaatgtgaaccacaagccttccaacaccaaggtggacaagagagtggaacccaagtcctgc

SEQ ID NO: 70 - DNA, 717 bp, synthetic construct
  misc_feature 1..717: note = source = /note="Description of Artificial Sequence: Synthetic polynucleotide"
  source 1..717: mol_type = other DNA
accatcaagccttgtcctccatgcaagtgccccgctcctaatctgctcggaggcccttccgtgttcatcttcccacctaagatcaaggacgtgctgatgatctccctgtctcctatcgtgacctgcgtggtggtggacgtgtccgaggatgatcctgacgtgcagatcagttggttcgtgaacaacgtggaagtgcacaccgctcagacccagacacacagagaggactacaacagcaccctgagagtggtgtctgccctgcctatccagcaccaggattggatgtccggcaaagaattcaagtgcaaagtgaacaacaaggacctgcctgctccaatcgagcggaccatctccaagcctggtggcggaaagcctaacatccagaatcctgagcctgccgtgtaccagctgaaggaccctagatctcaggactctaccctgtgcctgttcaccgacttcgactcccagatcaacgtgcccaagaccatggaatccggcaccttcatcaccgataagtgcgtgctggacatgaaggccatggactccaagtccaacggcgctatcgcctggtccaaccagaccagcttcacatgccaggacatcttcaaagagacaaacgccacctatccttccagcgacgtgccctgtgatgctaccctgaccgagaagtccttcgagacagacatgaacctgaacttccagaacctgtcctgatga

SEQ ID NO: 71 - DNA, 720 bp, synthetic construct
  misc_feature 1..720: note = source = /note="Description of Artificial Sequence: Synthetic polynucleotide"
  source 1..720: mol_type = other DNA
accatcaagccttgtcctccatgcaagtgccccgctcctaatctgctcggaggcccttccgtgttcatcttcccacctaagatcaaggacgtgctgatgatctccctgtctcctatcgtgacctgcgtggtggtggacgtgtccgaggatgatcctgacgtgcagatcagttggttcgtgaacaacgtggaagtgcacaccgctcagacccagacacacagagaggactacaacagcaccctgagagtggtgtctgccctgcctatccagcaccaggattggatgtccggcaaagaattcaagtgcaaagtgaacaacaaggacctgcctgctccaatcgagcggaccatctccaagcctggtggcggaggaaagcctaacatccagaatcctgagcctgccgtgtaccagctgaaggaccctagatctcaggactctaccctgtgcctgttcaccgacttcgactcccagatcaacgtgcccaagaccatggaatccggcaccttcatcaccgataagtgcgtgctggacatgaaggccatggactccaagtccaacggcgctatcgcctggtccaaccagaccagcttcacatgccaggacatcttcaaagagacaaacgccacctatccttccagcgacgtgccctgtgatgctaccctgaccgagaagtccttcgagacagacatgaacctgaacttccagaacctgtcctgatga

SEQ ID NO: 72 - DNA, 723 bp, synthetic construct
  misc_feature 1..723: note = source = /note="Description of Artificial Sequence: Synthetic polynucleotide"
  source 1..723: mol_type = other DNA
accatcaagccttgtcctccatgcaagtgccccgctcctaatctgctcggaggcccttccgtgttcatcttcccacctaagatcaaggacgtgctgatgatctccctgtctcctatcgtgacctgcgtggtggtggacgtgtccgaggatgatcctgacgtgcagatcagttggttcgtgaacaacgtggaagtgcacaccgctcagacccagacacacagagaggactacaacagcaccctgagagtggtgtctgccctgcctatccagcaccaggattggatgtccggcaaagaattcaagtgcaaagtgaacaacaaggacctgcctgctccaatcgagcggaccatctccaagcctggtggcggaggaagcaagcctaacatccagaatcctgagcctgccgtgtaccagctgaaggaccctagatctcaggactctaccctgtgcctgttcaccgacttcgactcccagatcaacgtgcccaagaccatggaatccggcaccttcatcaccgataagtgcgtgctggacatgaaggccatggactccaagtccaacggcgctatcgcctggtccaaccagaccagcttcacatgccaggacatcttcaaagagacaaacgccacctatccttccagcgacgtgccctgtgatgctaccctgaccgagaagtccttcgagacagacatgaacctgaacttccagaacctgtcctgatga

SEQ ID NO: 73 - DNA, 726 bp, synthetic construct
  misc_feature 1..726: note = source = /note="Description of Artificial Sequence: Synthetic polynucleotide"
  source 1..726: mol_type = other DNA
accatcaagccttgtcctccatgcaagtgccccgctcctaatctgctcggaggcccttccgtgttcatcttcccacctaagatcaaggacgtgctgatgatctccctgtctcctatcgtgacctgcgtggtggtggacgtgtccgaggatgatcctgacgtgcagatcagttggttcgtgaacaacgtggaagtgcacaccgctcagacccagacacacagagaggactacaacagcaccctgagagtggtgtctgccctgcctatccagcaccaggattggatgtccggcaaagaattcaagtgcaaagtgaacaacaaggacctgcctgctccaatcgagcggaccatctccaagcctggtggcggaggaagcggtaagcctaacatccagaatcctgagcctgccgtgtaccagctgaaggaccctagatctcaggactctaccctgtgcctgttcaccgacttcgactcccagatcaacgtgcccaagaccatggaatccggcaccttcatcaccgataagtgcgtgctggacatgaaggccatggactccaagtccaacggcgctatcgcctggtccaaccagaccagcttcacatgccaggacatcttcaaagagacaaacgccacctatccttccagcgacgtgccctgtgatgctaccctgaccgagaagtccttcgagacagacatgaacctgaacttccagaacctgtcctgatga

SEQ ID NO: 74 - DNA, 729 bp, synthetic construct
  misc_feature 1..729: note = source = /note="Description of Artificial Sequence: Synthetic polynucleotide"
  source 1..729: mol_type = other DNA
accatcaagccttgtcctccatgcaagtgccccgctcctaatctgctcggaggcccttccgtgttcatcttcccacctaagatcaaggacgtgctgatgatctccctgtctcctatcgtgacctgcgtggtggtggacgtgtccgaggatgatcctgacgtgcagatcagttggttcgtgaacaacgtggaagtgcacaccgctcagacccagacacacagagaggactacaacagcaccctgagagtggtgtctgccctgcctatccagcaccaggattggatgtccggcaaagaattcaagtgcaaagtgaacaacaaggacctgcctgctccaatcgagcggaccatctccaagcctggtggcggaggaagcggtggcaagcctaacatccagaatcctgagcctgccgtgtaccagctgaaggaccctagatctcaggactctaccctgtgcctgttcaccgacttcgactcccagatcaacgtgcccaagaccatggaatccggcaccttcatcaccgataagtgcgtgctggacatgaaggccatggactccaagtccaacggcgctatcgcctggtccaaccagaccagcttcacatgccaggacatcttcaaagagacaaacgccacctatccttccagcgacgtgccctgtgatgctaccctgaccgagaagtccttcgagacagacatgaacctgaacttccagaacctgtcctgatga

SEQ ID NO: 75 - DNA, 732 bp, synthetic construct
  misc_feature 1..732: note = source = /note="Description of Artificial Sequence: Synthetic polynucleotide"
  source 1..732: mol_type = other DNA
accatcaagccttgtcctccatgcaagtgccccgctcctaatctgctcggaggcccttccgtgttcatcttcccacctaagatcaaggacgtgctgatgatctccctgtctcctatcgtgacctgcgtggtggtggacgtgtccgaggatgatcctgacgtgcagatcagttggttcgtgaacaacgtggaagtgcacaccgctcagacccagacacacagagaggactacaacagcaccctgagagtggtgtctgccctgcctatccagcaccaggattggatgtccggcaaagaattcaagtgcaaagtgaacaacaaggacctgcctgctccaatcgagcggaccatctccaagcctggtggcggaggaagcggtggcggcaagcctaacatccagaatcctgagcctgccgtgtaccagctgaaggaccctagatctcaggactctaccctgtgcctgttcaccgacttcgactcccagatcaacgtgcccaagaccatggaatccggcaccttcatcaccgataagtgcgtgctggacatgaaggccatggactccaagtccaacggcgctatcgcctggtccaaccagaccagcttcacatgccaggacatcttcaaagagacaaacgccacctatccttccagcgacgtgccctgtgatgctaccctgaccgagaagtccttcgagacagacatgaacctgaacttccagaacctgtcctgatga

SEQ ID NO: 76 - DNA, 735 bp, synthetic construct
  misc_feature 1..735: note = source = /note="Description of Artificial Sequence: Synthetic polynucleotide"
  source 1..735: mol_type = other DNA
accatcaagccttgtcctccatgcaagtgccccgctcctaatctgctcggaggcccttccgtgttcatcttcccacctaagatcaaggacgtgctgatgatctccctgtctcctatcgtgacctgcgtggtggtggacgtgtccgaggatgatcctgacgtgcagatcagttggttcgtgaacaacgtggaagtgcacaccgctcagacccagacacacagagaggactacaacagcaccctgagagtggtgtctgccctgcctatccagcaccaggattggatgtccggcaaagaattcaagtgcaaagtgaacaacaaggacctgcctgctccaatcgagcggaccatctccaagcctggtggcggaggaagcggtggcggcggaaagcctaacatccagaatcctgagcctgccgtgtaccagctgaaggaccctagatctcaggactctaccctgtgcctgttcaccgacttcgactcccagatcaacgtgcccaagaccatggaatccggcaccttcatcaccgataagtgcgtgctggacatgaaggccatggactccaagtccaacggcgctatcgcctggtccaaccagaccagcttcacatgccaggacatcttcaaagagacaaacgccacctatccttccagcgacgtgccctgtgatgctaccctgaccgagaagtccttcgagacagacatgaacctgaacttccagaacctgtcctgatga

SEQ ID NO: 77 - DNA, 738 bp, synthetic construct
  misc_feature 1..738: note = source = /note="Description of Artificial Sequence: Synthetic polynucleotide"
  source 1..738: mol_type = other DNA
accatcaagccttgtcctccatgcaagtgccccgctcctaatctgctcggaggcccttccgtgttcatcttcccacctaagatcaaggacgtgctgatgatctccctgtctcctatcgtgacctgcgtggtggtggacgtgtccgaggatgatcctgacgtgcagatcagttggttcgtgaacaacgtggaagtgcacaccgctcagacccagacacacagagaggactacaacagcaccctgagagtggtgtctgccctgcctatccagcaccaggattggatgtccggcaaagaattcaagtgcaaagtgaacaacaaggacctgcctgctccaatcgagcggaccatctccaagcctggtggcggaggaagcggtggcggcggatctaagcctaacatccagaatcctgagcctgccgtgtaccagctgaaggaccctagatctcaggactctaccctgtgcctgttcaccgacttcgactcccagatcaacgtgcccaagaccatggaatccggcaccttcatcaccgataagtgcgtgctggacatgaaggccatggactccaagtccaacggcgctatcgcctggtccaaccagaccagcttcacatgccaggacatcttcaaagagacaaacgccacctatccttccagcgacgtgccctgtgatgctaccctgaccgagaagtccttcgagacagacatgaacctgaacttccagaacctgtcctgatga

SEQ ID NO: 78 - DNA, 1167 bp, synthetic construct
  misc_feature 1..1167: note = source = /note="Description of Artificial Sequence: Synthetic polynucleotide"
  source 1..1167: mol_type = other DNA
accatcaagccttgtcctccatgcaagtgccccgctcctaatctgctcggaggcccttccgtgttcatcttcccacctaagatcaaggacgtgctgatgatctccctgtctcctatcgtgacctgcgtggtggtggacgtgtccgaggatgatcctgacgtgcagatcagttggttcgtgaacaacgtggaagtgcacaccgctcagacccagacacacagagaggactacaacagcaccctgagagtggtgtctgccctgcctatccagcaccaggattggatgtccggcaaagaattcaagtgcaaagtgaacaacaaggacctgcctgctccaatcgagcggaccatctccaagcctgtggtggaagatctgcggaacgtgacccctcctaaggtgtccctgttcgagccttccaaggccgagatcgccaacaagcagaaagctaccctcgtgtgcctggccagaggcttctttcctgaccacgtggaactgtcttggtgggtcaacggcaaagaggtgcactccggcgtctgtaccgatcctcaggcctacaaagagtccaactactcctacagcctgtcctctcggctgagagtgtctgccaccttctggcacaaccctcggaaccacttcagatgccaggtgcagtttcacggcctgtccgaagaggacaagtggcctgagggatcccctaagcctgtgacacagaacatctctgccgaggcctggggtagagctgatggtggcggaggatctggcggaggtggaagcggcggaggcggatcttctcatctggaacagctgctgatggacctgcaagagctgctgtcccggatggaaaactaccggaacctgaagctgccccggatgctgaccgctaagttcgctctgcctaagcaggccaccgagctgaaggatctgcagtgcctggaagatgagctgggccctctgagacacgtgctggatctgacccagtccaagtcctttcagctcgaggacgccgagaacttcatctccaacatcagagtgaccgtggtcaagctgaagggctccgacaacaccttcgagtgccagttcgacgatgagtccgctacagtggtggacttcctgcggagatggatcgccttctgccagtccatcatctccacctctccacagtgatga

SEQ ID NO: 79 - DNA, 1170 bp, synthetic construct
  misc_feature 1..1170: note = source = /note="Description of Artificial Sequence: Synthetic polynucleotide"
  source 1..1170: mol_type = other DNA
accatcaagccttgtcctccatgcaagtgccccgctcctaatctgctcggaggcccttccgtgttcatcttcccacctaagatcaaggacgtgctgatgatctccctgtctcctatcgtgacctgcgtggtggtggacgtgtccgaggatgatcctgacgtgcagatcagttggttcgtgaacaacgtggaagtgcacaccgctcagacccagacacacagagaggactacaacagcaccctgagagtggtgtctgccctgcctatccagcaccaggattggatgtccggcaaagaattcaagtgcaaagtgaacaacaaggacctgcctgctccaatcgagcggaccatctccaagcctggtgtggtggaagatctgcggaacgtgacccctcctaaggtgtccctgttcgagccttccaaggccgagatcgccaacaagcagaaagctaccctcgtgtgcctggccagaggcttctttcctgaccacgtggaactgtcttggtgggtcaacggcaaagaggtgcactccggcgtctgtaccgatcctcaggcctacaaagagtccaactactcctacagcctgtcctctcggctgagagtgtctgccaccttctggcacaaccctcggaaccacttcagatgccaggtgcagtttcacggcctgtccgaagaggacaagtggcctgagggatcccctaagcctgtgacacagaacatctctgccgaggcctggggtagagctgatggtggcggaggatctggcggaggtggaagcggcggaggcggatcttctcatctggaacagctgctgatggacctgcaagagctgctgtcccggatggaaaactaccggaacctgaagctgccccggatgctgaccgctaagttcgctctgcctaagcaggccaccgagctgaaggatctgcagtgcctggaagatgagctgggccctctgagacacgtgctggatctgacccagtccaagtcctttcagctcgaggacgccgagaacttcatctccaacatcagagtgaccgtggtcaagctgaagggctccgacaacaccttcgagtgccagttcgacgatgagtccgctacagtggtggacttcctgcggagatggatcgccttctgccagtccatcatctccacctctccacagtgatga

SEQ ID NO: 80 - DNA, 1173 bp, synthetic construct
  misc_feature 1..1173: note = source = /note="Description of Artificial Sequence: Synthetic polynucleotide"
  source 1..1173: mol_type = other DNA
accatcaagccttgtcctccatgcaagtgccccgctcctaatctgctcggaggcccttccgtgttcatcttcccacctaagatcaaggacgtgctgatgatctccctgtctcctatcgtgacctgcgtggtggtggacgtgtccgaggatgatcctgacgtgcagatcagttggttcgtgaacaacgtggaagtgcacaccgctcagacccagacacacagagaggactacaacagcaccctgagagtggtgtctgccctgcctatccagcaccaggattggatgtccggcaaagaattcaagtgcaaagtgaacaacaaggacctgcctgctccaatcgagcggaccatctccaagcctggtggcgtggtggaagatctgcggaacgtgacccctcctaaggtgtccctgttcgagccttccaaggccgagatcgccaacaagcagaaagctaccctcgtgtgcctggccagaggcttctttcctgaccacgtggaactgtcttggtgggtcaacggcaaagaggtgcactccggcgtctgtaccgatcctcaggcctacaaagagtccaactactcctacagcctgtcctctcggctgagagtgtctgccaccttctggcacaaccctcggaaccacttcagatgccaggtgcagtttcacggcctgtccgaagaggacaagtggcctgagggatcccctaagcctgtgacacagaacatctctgccgaggcctggggtagagctgatggtggcggaggatctggcggaggtggaagcggcggaggcggatcttctcatctggaacagctgctgatggacctgcaagagctgctgtcccggatggaaaactaccggaacctgaagctgccccggatgctgaccgctaagttcgctctgcctaagcaggccaccgagctgaaggatctgcagtgcctggaagatgagctgggccctctgagacacgtgctggatctgacccagtccaagtcctttcagctcgaggacgccgagaacttcatctccaacatcagagtgaccgtggtcaagctgaagggctccgacaacaccttcgagtgccagttcgacgatgagtccgctacagtggtggacttcctgcggagatggatcgccttctgccagtccatcatctccacctctccacagtgatga

SEQ ID NO: 81 - DNA, 1176 bp, synthetic construct
  misc_feature 1..1176: note = source = /note="Description of Artificial Sequence: Synthetic polynucleotide"
  source 1..1176: mol_type = other DNA
accatcaagccttgtcctccatgcaagtgccccgctcctaatctgctcggaggcccttccgtgttcatcttcccacctaagatcaaggacgtgctgatgatctccctgtctcctatcgtgacctgcgtggtggtggacgtgtccgaggatgatcctgacgtgcagatcagttggttcgtgaacaacgtggaagtgcacaccgctcagacccagacacacagagaggactacaacagcaccctgagagtggtgtctgccctgcctatccagcaccaggattggatgtccggcaaagaattcaagtgcaaagtgaacaacaaggacctgcctgctccaatcgagcggaccatctccaagcctggtggcggagtggtggaagatctgcggaacgtgacccctcctaaggtgtccctgttcgagccttccaaggccgagatcgccaacaagcagaaagctaccctcgtgtgcctggccagaggcttctttcctgaccacgtggaactgtcttggtgggtcaacggcaaagaggtgcactccggcgtctgtaccgatcctcaggcctacaaagagtccaactactcctacagcctgtcctctcggctgagagtgtctgccaccttctggcacaaccctcggaaccacttcagatgccaggtgcagtttcacggcctgtccgaagaggacaagtggcctgagggatcccctaagcctgtgacacagaacatctctgccgaggcctggggtagagctgatggtggcggaggatctggcggaggtggaagcggcggaggcggatcttctcatctggaacagctgctgatggacctgcaagagctgctgtcccggatggaaaactaccggaacctgaagctgccccggatgctgaccgctaagttcgctctgcctaagcaggccaccgagctgaaggatctgcagtgcctggaagatgagctgggccctctgagacacgtgctggatctgacccagtccaagtcctttcagctcgaggacgccgagaacttcatctccaacatcagagtgaccgtggtcaagctgaagggctccgacaacaccttcgagtgccagttcgacgatgagtccgctacagtggtggacttcctgcggagatggatcgccttctgccagtccatcatctccacctctccacagtgatga

SEQ ID NO: 82 - DNA, 1179 bp, synthetic construct
  misc_feature 1..1179: note = source = /note="Description of Artificial Sequence: Synthetic polynucleotide"
  source 1..1179: mol_type = other DNA
accatcaagccttgtcctccatgcaagtgccccgctcctaatctgctcggaggcccttccgtgttcatcttcccacctaagatcaaggacgtgctgatgatctccctgtctcctatcgtgacctgcgtggtggtggacgtgtccgaggatgatcctgacgtgcagatcagttggttcgtgaacaacgtggaagtgcacaccgctcagacccagacacacagagaggactacaacagcaccctgagagtggtgtctgccctgcctatccagcaccaggattggatgtccggcaaagaattcaagtgcaaagtgaacaacaaggacctgcctgctccaatcgagcggaccatctccaagcctggtggcggaggagtggtggaagatctgcggaacgtgacccctcctaaggtgtccctgttcgagccttccaaggccgagatcgccaacaagcagaaagctaccctcgtgtgcctggccagaggcttctttcctgaccacgtggaactgtcttggtgggtcaacggcaaagaggtgcactccggcgtctgtaccgatcctcaggcctacaaagagtccaactactcctacagcctgtcctctcggctgagagtgtctgccaccttctggcacaaccctcggaaccacttcagatgccaggtgcagtttcacggcctgtccgaagaggacaagtggcctgagggatcccctaagcctgtgacacagaacatctctgccgaggcctggggtagagctgatggtggcggaggatctggcggaggtggaagcggcggaggcggatcttctcatctggaacagctgctgatggacctgcaagagctgctgtcccggatggaaaactaccggaacctgaagctgccccggatgctgaccgctaagttcgctctgcctaagcaggccaccgagctgaaggatctgcagtgcctggaagatgagctgggccctctgagacacgtgctggatctgacccagtccaagtcctttcagctcgaggacgccgagaacttcatctccaacatcagagtgaccgtggtcaagctgaagggctccgacaacaccttcgagtgccagttcgacgatgagtccgctacagtggtggacttcctgcggagatggatcgccttctgccagtccatcatctccacctctccacagtgatga

SEQ ID NO: 83 - DNA, 1182 bp, synthetic construct
  misc_feature 1..1182: note = source = /note="Description of Artificial Sequence: Synthetic polynucleotide"
  source 1..1182: mol_type = other DNA
accatcaagccttgtcctccatgcaagtgccccgctcctaatctgctcggaggcccttccgtgttcatcttcccacctaagatcaaggacgtgctgatgatctccctgtctcctatcgtgacctgcgtggtggtggacgtgtccgaggatgatcctgacgtgcagatcagttggttcgtgaacaacgtggaagtgcacaccgctcagacccagacacacagagaggactacaacagcaccctgagagtggtgtctgccctgcctatccagcaccaggattggatgtccggcaaagaattcaagtgcaaagtgaacaacaaggacctgcctgctccaatcgagcggaccatctccaagcctggtggcggaggaagcgtggtggaagatctgcggaacgtgacccctcctaaggtgtccctgttcgagccttccaaggccgagatcgccaacaagcagaaagctaccctcgtgtgcctggccagaggcttctttcctgaccacgtggaactgtcttggtgggtcaacggcaaagaggtgcactccggcgtctgtaccgatcctcaggcctacaaagagtccaactactcctacagcctgtcctctcggctgagagtgtctgccaccttctggcacaaccctcggaaccacttcagatgccaggtgcagtttcacggcctgtccgaagaggacaagtggcctgagggatcccctaagcctgtgacacagaacatctctgccgaggcctggggtagagctgatggtggcggaggatctggcggaggtggaagcggcggaggcggatcttctcatctggaacagctgctgatggacctgcaagagctgctgtcccggatggaaaactaccggaacctgaagctgccccggatgctgaccgctaagttcgctctgcctaagcaggccaccgagctgaaggatctgcagtgcctggaagatgagctgggccctctgagacacgtgctggatctgacccagtccaagtcctttcagctcgaggacgccgagaacttcatctccaacatcagagtgaccgtggtcaagctgaagggctccgacaacaccttcgagtgccagttcgacgatgagtccgctacagtggtggacttcctgcggagatggatcgccttctgccagtccatcatctccacctctccacagtgatga

SEQ ID NO: 84 - DNA, 1185 bp, synthetic construct
  misc_feature 1..1185: note = source = /note="Description of Artificial Sequence: Synthetic polynucleotide"
  source 1..1185: mol_type = other DNA
accatcaagccttgtcctccatgcaagtgccccgctcctaatctgctcggaggcccttccgtgttcatcttcccacctaagatcaaggacgtgctgatgatctccctgtctcctatcgtgacctgcgtggtggtggacgtgtccgaggatgatcctgacgtgcagatcagttggttcgtgaacaacgtggaagtgcacaccgctcagacccagacacacagagaggactacaacagcaccctgagagtggtgtctgccctgcctatccagcaccaggattggatgtccggcaaagaattcaagtgcaaagtgaacaacaaggacctgcctgctccaatcgagcggaccatctccaagcctggtggcggaggaagcggtgtggtggaagatctgcggaacgtgacccctcctaaggtgtccctgttcgagccttccaaggccgagatcgccaacaagcagaaagctaccctcgtgtgcctggccagaggcttctttcctgaccacgtggaactgtcttggtgggtcaacggcaaagaggtgcactccggcgtctgtaccgatcctcaggcctacaaagagtccaactactcctacagcctgtcctctcggctgagagtgtctgccaccttctggcacaaccctcggaaccacttcagatgccaggtgcagtttcacggcctgtccgaagaggacaagtggcctgagggatcccctaagcctgtgacacagaacatctctgccgaggcctggggtagagctgatggtggcggaggatctggcggaggtggaagcggcggaggcggatcttctcatctggaacagctgctgatggacctgcaagagctgctgtcccggatggaaaactaccggaacctgaagctgccccggatgctgaccgctaagttcgctctgcctaagcaggccaccgagctgaaggatctgcagtgcctggaagatgagctgggccctctgagacacgtgctggatctgacccagtccaagtcctttcagctcgaggacgccgagaacttcatctccaacatcagagtgaccgtggtcaagctgaagggctccgacaacaccttcgagtgccagttcgacgatgagtccgctacagtggtggacttcctgcggagatggatcgccttctgccagtccatcatctccacctctccacagtgatga

SEQ ID NO: 85 - DNA, 1188 bp, synthetic construct
  misc_feature 1..1188: note = source = /note="Description of Artificial Sequence: Synthetic polynucleotide"
  source 1..1188: mol_type = other DNA
accatcaagccttgtcctccatgcaagtgccccgctcctaatctgctcggaggcccttccgtgttcatcttcccacctaagatcaaggacgtgctgatgatctccctgtctcctatcgtgacctgcgtggtggtggacgtgtccgaggatgatcctgacgtgcagatcagttggttcgtgaacaacgtggaagtgcacaccgctcagacccagacacacagagaggactacaacagcaccctgagagtggtgtctgccctgcctatccagcaccaggattggatgtccggcaaagaattcaagtgcaaagtgaacaacaaggacctgcctgctccaatcgagcggaccatctccaagcctggtggcggaggaagcggtggcgtggtggaagatctgcggaacgtgacccctcctaaggtgtccctgttcgagccttccaaggccgagatcgccaacaagcagaaagctaccctcgtgtgcctggccagaggcttctttcctgaccacgtggaactgtcttggtgggtcaacggcaaagaggtgcactccggcgtctgtaccgatcctcaggcctacaaagagtccaactactcctacagcctgtcctctcggctgagagtgtctgccaccttctggcacaaccctcggaaccacttcagatgccaggtgcagtttcacggcctgtccgaagaggacaagtggcctgagggatcccctaagcctgtgacacagaacatctctgccgaggcctggggtagagctgatggtggcggaggatctggcggaggtggaagcggcggaggcggatcttctcatctggaacagctgctgatggacctgcaagagctgctgtcccggatggaaaactaccggaacctgaagctgccccggatgctgaccgctaagttcgctctgcctaagcaggccaccgagctgaaggatctgcagtgcctggaagatgagctgggccctctgagacacgtgctggatctgacccagtccaagtcctttcagctcgaggacgccgagaacttcatctccaacatcagagtgaccgtggtcaagctgaagggctccgacaacaccttcgagtgccagttcgacgatgagtccgctacagtggtggacttcctgcggagatggatcgccttctgccagtccatcatctccacctctccacagtgatga

SEQ ID NO: 86 - DNA, 1191 bp, synthetic construct
  misc_feature 1..1191: note = source = /note="Description of Artificial Sequence: Synthetic polynucleotide"
  source 1..1191: mol_type = other DNA
accatcaagccttgtcctccatgcaagtgccccgctcctaatctgctcggaggcccttccgtgttcatcttcccacctaagatcaaggacgtgctgatgatctccctgtctcctatcgtgacctgcgtggtggtggacgtgtccgaggatgatcctgacgtgcagatcagttggttcgtgaacaacgtggaagtgcacaccgctcagacccagacacacagagaggactacaacagcaccctgagagtggtgtctgccctgcctatccagcaccaggattggatgtccggcaaagaattcaagtgcaaagtgaacaacaaggacctgcctgctccaatcgagcggaccatctccaagcctggtggcggaggaagcggtggcggcgtggtggaagatctgcggaacgtgacccctcctaaggtgtccctgttcgagccttccaaggccgagatcgccaacaagcagaaagctaccctcgtgtgcctggccagaggcttctttcctgaccacgtggaactgtcttggtgggtcaacggcaaagaggtgcactccggcgtctgtaccgatcctcaggcctacaaagagtccaactactcctacagcctgtcctctcggctgagagtgtctgccaccttctggcacaaccctcggaaccacttcagatgccaggtgcagtttcacggcctgtccgaagaggacaagtggcctgagggatcccctaagcctgtgacacagaacatctctgccgaggcctggggtagagctgatggtggcggaggatctggcggaggtggaagcggcggaggcggatcttctcatctggaacagctgctgatggacctgcaagagctgctgtcccggatggaaaactaccggaacctgaagctgccccggatgctgaccgctaagttcgctctgcctaagcaggccaccgagctgaaggatctgcagtgcctggaagatgagctgggccctctgagacacgtgctggatctgacccagtccaagtcctttcagctcgaggacgccgagaacttcatctccaacatcagagtgaccgtggtcaagctgaagggctccgacaacaccttcgagtgccagttcgacgatgagtccgctacagtggtggacttcctgcggagatggatcgccttctgccagtccatcatctccacctctccacagtgatga

SEQ ID NO: 87 - DNA, 1194 bp, synthetic construct
  misc_feature 1..1194: note = source = /note="Description of Artificial Sequence: Synthetic polynucleotide"
  source 1..1194: mol_type = other DNA
accatcaagccttgtcctccatgcaagtgccccgctcctaatctgctcggaggcccttccgtgttcatcttcccacctaagatcaaggacgtgctgatgatctccctgtctcctatcgtgacctgcgtggtggtggacgtgtccgaggatgatcctgacgtgcagatcagttggttcgtgaacaacgtggaagtgcacaccgctcagacccagacacacagagaggactacaacagcaccctgagagtggtgtctgccctgcctatccagcaccaggattggatgtccggcaaagaattcaagtgcaaagtgaacaacaaggacctgcctgctccaatcgagcggaccatctccaagcctggtggcggaggaagcggtggcggcggagtggtggaagatctgcggaacgtgacccctcctaaggtgtccctgttcgagccttccaaggccgagatcgccaacaagcagaaagctaccctcgtgtgcctggccagaggcttctttcctgaccacgtggaactgtcttggtgggtcaacggcaaagaggtgcactccggcgtctgtaccgatcctcaggcctacaaagagtccaactactcctacagcctgtcctctcggctgagagtgtctgccaccttctggcacaaccctcggaaccacttcagatgccaggtgcagtttcacggcctgtccgaagaggacaagtggcctgagggatcccctaagcctgtgacacagaacatctctgccgaggcctggggtagagctgatggtggcggaggatctggcggaggtggaagcggcggaggcggatcttctcatctggaacagctgctgatggacctgcaagagctgctgtcccggatggaaaactaccggaacctgaagctgccccggatgctgaccgctaagttcgctctgcctaagcaggccaccgagctgaaggatctgcagtgcctggaagatgagctgggccctctgagacacgtgctggatctgacccagtccaagtcctttcagctcgaggacgccgagaacttcatctccaacatcagagtgaccgtggtcaagctgaagggctccgacaacaccttcgagtgccagttcgacgatgagtccgctacagtggtggacttcctgcggagatggatcgccttctgccagtccatcatctccacctctccacagtgatga

SEQ ID NO: 88 - DNA, 1197 bp, synthetic construct
  misc_feature 1..1197: note = source = /note="Description of Artificial Sequence: Synthetic polynucleotide"
  source 1..1197: mol_type = other DNA
accatcaagccttgtcctccatgcaagtgccccgctcctaatctgctcggaggcccttccgtgttcatcttcccacctaagatcaaggacgtgctgatgatctccctgtctcctatcgtgacctgcgtggtggtggacgtgtccgaggatgatcctgacgtgcagatcagttggttcgtgaacaacgtggaagtgcacaccgctcagacccagacacacagagaggactacaacagcaccctgagagtggtgtctgccctgcctatccagcaccaggattggatgtccggcaaagaattcaagtgcaaagtgaacaacaaggacctgcctgctccaatcgagcggaccatctccaagcctggtggcggaggaagcggtggcggcggatctgtggtggaagatctgcggaacgtgacccctcctaaggtgtccctgttcgagccttccaaggccgagatcgccaacaagcagaaagctaccctcgtgtgcctggccagaggcttctttcctgaccacgtggaactgtcttggtgggtcaacggcaaagaggtgcactccggcgtctgtaccgatcctcaggcctacaaagagtccaactactcctacagcctgtcctctcggctgagagtgtctgccaccttctggcacaaccctcggaaccacttcagatgccaggtgcagtttcacggcctgtccgaagaggacaagtggcctgagggatcccctaagcctgtgacacagaacatctctgccgaggcctggggtagagctgatggtggcggaggatctggcggaggtggaagcggcggaggcggatcttctcatctggaacagctgctgatggacctgcaagagctgctgtcccggatggaaaactaccggaacctgaagctgccccggatgctgaccgctaagttcgctctgcctaagcaggccaccgagctgaaggatctgcagtgcctggaagatgagctgggccctctgagacacgtgctggatctgacccagtccaagtcctttcagctcgaggacgccgagaacttcatctccaacatcagagtgaccgtggtcaagctgaagggctccgacaacaccttcgagtgccagttcgacgatgagtccgctacagtggtggacttcctgcggagatggatcgccttctgccagtccatcatctccacctctccacagtgatga

SEQ ID NO: 89 - DNA, 1344 bp, synthetic construct
  misc_feature 1..1344: note = source = /note="Description of Artificial Sequence: Synthetic polynucleotide"
  source 1..1344: mol_type = other DNA
caggtgcagctggtggaatctggtggcggagttgtgcagcctggcagatccctgagactgtcttgtgccgcctccggcttcaccttctccagctacaccatgcactgggtccgacaggcccctggcaaaggattggagtgggtcaccttcatctcttacgacggcaacaacaagtactacgccgactccgtgaagggcagattcaccatctctcgggacaactccaagaacaccctgtacctgcagatgaactccctgagagccgaggacaccgccatctactactgtgctagaaccggctggctgggcccctttgattattggggacagggcaccctggtcaccgtgtcctctgcttccaccaagggaccctctgtgttccctctggctccttccagcaagtctacctctggcggaacagctgctctgggctgcctggtcaaggactactttcctgagcctgtgaccgtgtcttggaactctggcgctctgacatccggcgtgcacacctttccagctgtgctgcaatcctccggcctgtactctctgtcctccgtcgtgaccgtgccttctagctctctgggcacccagacctacatctgcaatgtgaaccacaagccttccaacaccaaggtggacaagagagtggaacccaagtcctgcgataagacccacacctgtccaccatgtcctgctccagaactgctcggcggaccttccgtgttcctgtttcctccaaagcctaaggacaccctgatgatctctcggacccctgaagtgacctgcgtggtggtggatgtgtctcacgaggatcccgaagtgaagttcaattggtacgtggacggcgtggaagtgcacaacgccaagaccaagcctagagaggaacagtacaactccacctacagagtggtgtccgtgctgaccgtgctgcaccaggattggctgaacggcaaagagtacaagtgcaaggtgtccaacaaggccctgcctgctcctatcgaaaagaccatctccaaggccaaaggccagcctagggaaccccaggtttacaccctgcctccatgccgggaagagatgaccaagaaccaggtgtccctgtggtgcctggttaagggcttctacccctccgatatcgccgtggaatgggagtctaatggccagcctgagaacaactacaagacaacccctcctgtgctggactccgacggctcattcttcctgtactccaagctgacagtggacaagtccagatggcagcagggcaacgtgttctcctgctccgtgatgcacgaggccctgcacaatcactacacccagaagtccctgtctctgagccccggcaag

SEQ ID NO: 90 - DNA, 1334 bp, synthetic construct
  misc_feature 1..1334: note = source = /note="Description of Artificial Sequence: Synthetic polynucleotide"
  source 1..1334: mol_type = other DNA
caggtgcagctggtggaatctggtggcggagttgtgcagcctggcagatccctgagactgtcttgtgccgcctccggcttcaccttctcctcttacggaatgcactgggtccgacaggcccctggcaaaggattggagtgggtcgccttcatcagatacgacggctccaacaagtactacgccgactccgtgaagggcagattcaccatctctcgggacaactccaagaacaccctgtacctgcagatgaactccctgagagccgaggacaccgccgtgtactactgcaagacccacggctctcacgacaattggggccagggcacaatggtcaccgtgtcctctgcttccaccaagggaccctctgtgttccctctggctccttccagcaagtctacctctggcggaacagctgctctgggctgcctggtcaaggactactttcctgagcctgtgaccgtgtcttggaactctggcgctctgacatccggcgtgcacacctttccagctgtgctgcaatcctccggcctgtactctctgtcctccgtcgtgaccgtgccttctagctctctgggcacccagacctacatctgcaatgtgaaccacaagccttccaacaccaaggtggacaagagagtggaacccaagtcctgcgataagacccacacctgtccaccatgtcctgctccagaactgctcggcggaccttccgtgttcctgtttcctccaaagcctaaggacaccctgatgatctctcggacccctgaagtgacctgcgtggtggtggatgtgtctcacgaggatcccgaagtgaagttcaattggtacgtggacggcgtggaagtgcacaacgccaagaccaagcctagagaggaacagtacaactccacctacagagtggtgtccgtgctgaccgtgctgcaccaggattggctgaacggcaaagagtacaagtgcaaggtgtccaacaaggccctgcctgctcctatcgaaaagaccatctccaaggccaaagccagcctcgggaacctcaagtctgtaccctgcctcctagccgggaagagatgaccaagaaccaggtgtccctgtcctgcgctgtgaagggcttctacccttccgatatcgccgtggaatgggagagcaatggccagcctgagaacaactacaagaccacacctcctgtgctggactccgacggctcattcttcctggtgtccaagctgacagtggacaagtccagatggcagcagggcaacgtgttctcctgctccgtgatgcacgaggccctgcacaatcactacacccagaagtccctgtctctgagccccggcaag

SEQ ID NO: 91 - protein, 118 aa, synthetic construct
  REGION 1..118: note = source = /note="Description of Artificial Sequence: Synthetic polypeptide"
QVQLVESGGGVVQPGRSLRLSCAASGFTFSSYTMHWVRQAPGKGLEWVTFISYDGNNKYYADSVKGRFTISRDNSKNTLYLQMNSLRAEDTAIYYCARTGWLGPFDYWGQGTLVTVSS

SEQ ID NO: 92 - protein, 108 aa, synthetic construct
  REGION 1..108: note = source = /note="Description of Artificial Sequence: Synthetic polypeptide"
EIVLTQSPGTLSLSPGERATLSCRASQSVGSSYLAWYQQKPGQAPRLLIYGAFSRATGIPDRFSGSGSGTDFTLTISRLEPEDFAVYYCQQYGSSPWTFGQGTKVEIK

SEQ ID NO: 93 - protein, 115 aa, synthetic construct [sequence omitted]

SEQ ID NO: 94 - protein, 111 aa, synthetic construct [sequence omitted]

SEQ ID NO: 95 - protein, 107 aa, synthetic construct [sequence omitted]

SEQ ID NO: 96 - protein, 106 aa, synthetic construct
  REGION 1..106: note = source = /note="Description of Artificial Sequence: Synthetic polypeptide"
GQPKANPTVTLFPPSSEELQANKATLVCLISDFYPGAVTVAWKADGSPVKAGVETTKPSKQSNNKYAASSYLSLTPEQWKSHRSYSCQVTHEGSTVEKTVAPTECS

SEQ ID NO: 97 - protein, 103 aa, synthetic construct
  REGION 1..103: note = source = /note="Description of Artificial Sequence: Synthetic polypeptide"
ASTKGPSVFPLAPSSKSTSGGTAALGCLVKDYFPEPVTVSWNSGALTSGVHTFPAVLQSSGLYSLSSVVTVPSSSLGTQTYICNVNHKPSNTKVDKRVEPKSC

SEQ ID NO: 98 - protein, 120 aa, synthetic construct
  REGION 1..120: note = source = /note="Description of Artificial Sequence: Synthetic polypeptide"
DKTHTCPPCPAPELLGGPSVFLFPPKPKDTLMISRTPEVTCVVVDVSHEDPEVKFNWYVDGVEVHNAKTKPREEQYNSTYRVVSVLTVLHQDWLNGKEYKCKVSNKALPAPIEKTISKAK

SEQ ID NO: 99 - protein, 93 aa, synthetic construct; identical to SEQ ID NO: 1
  REGION 1..93: note = source = /note="Description of Artificial Sequence: Synthetic polypeptide"

SEQ ID NO: 100 - protein, 130 aa, synthetic construct; identical to SEQ ID NO: 2
  REGION 1..130: note = source = /note="Description of Artificial Sequence: Synthetic polypeptide"

SEQ ID NO: 101-103 - skipped (3 entries)

SEQ ID NO: 104 - protein, 4 aa, synthetic construct
  REGION 1..4: note = source = /note="Description of Artificial Sequence: Synthetic peptide"
GGGG

SEQ ID NO: 105 - protein, 5 aa, synthetic construct
  REGION 1..5: note = source = /note="Description of Artificial Sequence: Synthetic peptide"
GGGGS

SEQ ID NO: 106 - protein, 6 aa, synthetic construct
  REGION 1..6: note = source = /note="Description of Artificial Sequence: Synthetic peptide"
GGGGSG

SEQ ID NO: 107 - protein, 7 aa, synthetic construct
  REGION 1..7: note = source = /note="Description of Artificial Sequence: Synthetic peptide"
GGGGSGG

SEQ ID NO: 108 - protein, 8 aa, synthetic construct
  REGION 1..8: note = source = /note="Description of Artificial Sequence: Synthetic peptide"
GGGGSGGG

SEQ ID NO: 109 - protein, 9 aa, synthetic construct
  REGION 1..9: note = source = /note="Description of Artificial Sequence: Synthetic peptide"
GGGGSGGGG

SEQ ID NO: 110 - protein, 10 aa, synthetic construct
  REGION 1..10: note = source = /note="Description of Artificial Sequence: Synthetic peptide"
GGGGSGGGGS

SEQ ID NO: 111 - protein, 120 aa, synthetic construct
  REGION 1..120: note = source = /note="Description of Artificial Sequence: Synthetic polypeptide"
TIKPCPPCKCPAPNLLGGPSVFIFPPKIKDVLMISLSPIVTCVVVDVSEDDPDVQISWFVNNVEVHTAQTQTHREDYNSTLRVVSALPIQHQDWMSGKEFKCKVNNKDLPAPIERTISKP

SEQ ID NO: 112 - protein, 114 aa, synthetic construct
  REGION 1..114: note = source = /note="Description of Artificial Sequence: Synthetic polypeptide"
KPNIQNPEPAVYQLKDPRSQDSTLCLFTDFDSQINVPKTMESGTFITDKCVLDMKAMDSKSNGAIAWSNQTSFTCQDIFKETNATYPSSDVPCDATLTEKSFETDMNLNFQNLS

SEQ ID NO: 113 - protein, 128 aa, synthetic construct
  REGION 1..128: note = source = /note="Description of Artificial Sequence: Synthetic polypeptide"
VVEDLRNVTPPKVSLFEPSKAEIANKQKATLVCLARGFFPDHVELSWWVNGKEVHSGVCTDPQAYKESNYSYSLSSRLRVSATFWHNPRNHFRCQVQFHGLSEEDKWPEGSPKPVTQNISAEAWGRAD

SEQ ID NO: 114 - protein, 124 aa, synthetic construct
  REGION 1..124: note = source = /note="Description of Artificial Sequence: Synthetic polypeptide"
SHLEQLLMDLQELLSRMENYRNLKLPRMLTAKFALPKQATELKDLQCLEDELGPLRHVLDLTQSKSFQLEDAENFISNIRVTVVKLKGSDNTFECQFDDESATVVDFLRRWIAFCQSIISTSPQ

SEQ ID NO: 115 - protein, 15 aa, synthetic construct
  REGION 1..15: note = source = /note="Description of Artificial Sequence: Synthetic peptide"
GGGGSGGGGSGGGGS

SEQ ID NO: 116 - protein, 107 aa, synthetic construct
  REGION 1..107: note = source = /note="Description of Artificial Sequence: Synthetic polypeptide"
GQPREPQVYTLPPCREEMTKNQVSLWCLVKGFYPSDIAVEWESNGQPENNYKTTPPVLDSDGSFFLYSKLTVDKSRWQQGNVFSCSVMHEALHNHYTQKSLSLSPGK

SEQ ID NO: 117 - protein, 107 aa, synthetic construct
  REGION 1..107: note = source = /note="Description of Artificial Sequence: Synthetic polypeptide"
GQPREPQVCTLPPSREEMTKNQVSLSCAVKGFYPSDIAVEWESNGQPENNYKTTPPVLDSDGSFFLVSKLTVDKSRWQQGNVFSCSVMHEALHNHYTQKSLSLSPGK

SEQ ID NO: 118 - protein, 434 aa, synthetic construct
  REGION 1..434: note = source = /note="Description of Artificial Sequence: Synthetic polypeptide"
QVQLVESGGGVVQPGRSLRLSCAASGFTFSSYTMHWVRQAPGKGLEWVTFISYDGNNKYYADSVKGRFTISRDNSKNTLYLQMNSLRAEDTAIYYCARTGWLGPFDYWGQGTLVTVSSASTKGPSVFPLAPSSKSTSGGTAALGCLVKDYFPEPVTVSWNSGALTSGVHTFPAVLQSSGLYSLSSVVTVPSSSLGTQTYICNVNHKPSNTKVDKRVEPKSCDKTHTCPPCPAPELLGGPSVFLFPPKPKDTLMISRTPEVTCVVVDVSHEDPEVKFNWYVDGVEVHNAKTKPREEQYNSTYRVVSVLTVLHQDWLNGKEYKCKVSNKALPAPIEKTISKAKPDIQNPDPAVYQLRDSKSSDKSVCLFTDFDSQTNVSQSKDSDVYITDKCVLDMRSMDFKSNSAVAWSNKSDFACANAFNNSIIPEDTFFPSPE

SEQ ID NO: 119 - protein, 435 aa, synthetic construct
  REGION 1..435: note = source = /note="Description of Artificial Sequence: Synthetic polypeptide"
QVQLVESGGGVVQPGRSLRLSCAASGFTFSSYTMHWVRQAPGKGLEWVTFISYDGNNKYYADSVKGRFTISRDNSKNTLYLQMNSLRAEDTAIYYCARTGWLGPFDYWGQGTLVTVSSASTKGPSVFPLAPSSKSTSGGTAALGCLVKDYFPEPVTVSWNSGALTSGVHTFPAVLQSSGLYSLSSVVTVPSSSLGTQTYICNVNHKPSNTKVDKRVEPKSCDKTHTCPPCPAPELLGGPSVFLFPPKPKDTLMISRTPEVTCVVVDVSHEDPEVKFNWYVDGVEVHNAKTKPREEQYNSTYRVVSVLTVLHQDWLNGKEYKCKVSNKALPAPIEKTISKAKGPDIQNPDPAVYQLRDSKSSDKSVCLFTDFDSQTNVSQSKDSDVYITDKCVLDMRSMDFKSNSAVAWSNKSDFACANAFNNSIIPEDTFFPSPE

SEQ ID NO: 120 - protein, 436 aa, synthetic construct
  REGION 1..436: note = source = /note="Description of Artificial Sequence: Synthetic polypeptide"
QVQLVESGGGVVQPGRSLRLSCAASGFTFSSYTMHWVRQAPGKGLEWVTFISYDGNNKYYADSVKGRFTISRDNSKNTLYLQMNSLRAEDTAIYYCARTGWLGPFDYWGQGTLVTVSSASTKGPSVFPLAPSSKSTSGGTAALGCLVKDYFPEPVTVSWNSGALTSGVHTFPAVLQSSGLYSLSSVVTVPSSSLGTQTYICNVNHKPSNTKVDKRVEPKSCDKTHTCPPCPAPELLGGPSVFLFPPKPKDTLMISRTPEVTCVVVDVSHEDPEVKFNWYVDGVEVHNAKTKPREEQYNSTYRVVSVLTVLHQDWLNGKEYKCKVSNKALPAPIEKTISKAKGGPDIQNPDPAVYQLRDSKSSDKSVCLFTDFDSQTNVSQSKDSDVYITDKCVLDMRSMDFKSNSAVAWSNKSDFACANAFNNSIIPEDTFFPSPE

SEQ ID NO: 121 - protein, 437 aa, synthetic construct
  REGION 1..437: note = source = /note="Description of Artificial Sequence: Synthetic polypeptide"
QVQLVESGGGVVQPGRSLRLSCAASGFTFSSYTMHWVRQAPGKGLEWVTFISYDGNNKYYADSVKGRFTISRDNSKNTLYLQMNSLRAEDTAIYYCARTGWLGPFDYWGQGTLVTVSSASTKGPSVFPLAPSSKSTSGGTAALGCLVKDYFPEPVTVSWNSGALTSGVHTFPAVLQSSGLYSLSSVVTVPSSSLGTQTYICNVNHKPSNTKVDKRVEPKSCDKTHTCPPCPAPELLGGPSVFLFPPKPKDTLMISRTPEVTCVVVDVSHEDPEVKFNWYVDGVEVHNAKTKPREEQYNSTYRVVSVLTVLHQDWLNGKEYKCKVSNKALPAPIEKTISKAKGGGPDIQNPDPAVYQLRDSKSSDKSVCLFTDFDSQTNVSQSKDSDVYITDKCVLDMRSMDFKSNSAVAWSNKSDFACANAFNNSIIPEDTFFPSPE

SEQ ID NO: 122 - protein, 438 aa, synthetic construct
  REGION 1..438: note = source = /note="Description of Artificial Sequence: Synthetic polypeptide"
QVQLVESGGGVVQPGRSLRLSCAASGFTFSSYTMHWVRQAPGKGLEWVTFISYDGNNKYYADSVKGRFTISRDNSKNTLYLQMNSLRAEDTAIYYCARTGWLGPFDYWGQGTLVTVSSASTKGPSVFPLAPSSKSTSGGTAALGCLVKDYFPEPVTVSWNSGALTSGVHTFPAVLQSSGLYSLSSVVTVPSSSLGTQTYICNVNHKPSNTKVDKRVEPKSCDKTHTCPPCPAPELLGGPSVFLFPPKPKDTLMISRTPEVTCVVVDVSHEDPEVKFNWYVDGVEVHNAKTKPREEQYNSTYRVVSVLTVLHQDWLNGKEYKCKVSNKALPAPIEKTISKAKGGGGPDIQNPDPAVYQLRDSKSSDKSVCLFTDFDSQTNVSQSKDSDVYITDKCVLDMRSMDFKSNSAVAWSNKSDFACANAFNNSIIPEDTFFPSPE

SEQ ID NO: 123 - protein, 439 aa, synthetic construct
  REGION 1..439: note = source = /note="Description of Artificial Sequence: Synthetic polypeptide"
QVQLVESGGGVVQPGRSLRLSCAASGFTFSSYTMHWVRQAPGKGLEWVTFISYDGNNKYYADSVKGRFTISRDNSKNTLYLQMNSLRAEDTAIYYCARTGWLGPFDYWGQGTLVTVSSASTKGPSVFPLAPSSKSTSGGTAALGCLVKDYFPEPVTVSWNSGALTSGVHTFPAVLQSSGLYSLSSVVTVPSSSLGTQTYICNVNHKPSNTKVDKRVEPKSCDKTHTCPPCPAPELLGGPSVFLFPPKPKDTLMISRTPEVTCVVVDVSHEDPEVKFNWYVDGVEVHNAKTKPREEQYNSTYRVVSVLTVLHQDWLNGKEYKCKVSNKALPAPIEKTISKAKGGGGSPDIQNPDPAVYQLRDSKSSDKSVCLFTDFDSQTNVSQSKDSDVYITDKCVLDMRSMDFKSNSAVAWSNKSDFACANAFNNSIIPEDTFFPSPE

SEQ ID NO: 124 - protein, 440 aa, synthetic construct
  REGION 1..440: note = source = /note="Description of Artificial Sequence: Synthetic polypeptide"
QVQLVESGGGVVQPGRSLRLSCAASGFTFSSYTMHWVRQAPGKGLEWVTFISYDGNNKYYADSVKGRFTISRDNSKNTLYLQMNSLRAEDTAIYYCARTGWLGPFDYWGQGTLVTVSSASTKGPSVFPLAPSSKSTSGGTAALGCLVKDYFPEPVTVSWNSGALTSGVHTFPAVLQSSGLYSLSSVVTVPSSSLGTQTYICNVNHKPSNTKVDKRVEPKSCDKTHTCPPCPAPELLGGPSVFLFPPKPKDTLMISRTPEVTCVVVDVSHEDPEVKFNWYVDGVEVHNAKTKPREEQYNSTYRVVSVLTVLHQDWLNGKEYKCKVSNKALPAPIEKTISKAKGGGGSGPDIQNPDPAVYQLRDSKSSDKSVCLFTDFDSQTNVSQSKDSDVYITDKCVLDMRSMDFKSNSAVAWSNKSDFACANAFNNSIIPEDTFFPSPE

SEQ ID NO: 125 - protein, 441 aa, synthetic construct
  REGION 1..441: note = source = /note="Description of Artificial Sequence: Synthetic polypeptide"
QVQLVESGGGVVQPGRSLRLSCAASGFTFSSYTMHWVRQAPGKGLEWVTFISYDGNNKYYADSVKGRFTISRDNSKNTLYLQMNSLRAEDTAIYYCARTGWLGPFDYWGQGTLVTVSSASTKGPSVFPLAPSSKSTSGGTAALGCLVKDYFPEPVTVSWNSGALTSGVHTFPAVLQSSGLYSLSSVVTVPSSSLGTQTYICNVNHKPSNTKVDKRVEPKSCDKTHTCPPCPAPELLGGPSVFLFPPKPKDTLMISRTPEVTCVVVDVSHEDPEVKFNWYVDGVEVHNAKTKPREEQYNSTYRVVSVLTVLHQDWLNGKEYKCKVSNKALPAPIEKTISKAKGGGGSGGPDIQNPDPAVYQLRDSKSSDKSVCLFTDFDSQTNVSQSKDSDVYITDKCVLDMRSMDFKSNSAVAWSNKSDFACANAFNNSIIPEDTFFPSPE

SEQ ID NO: 126 - protein, 442 aa, synthetic construct
  REGION 1..442: note = source = /note="Description of Artificial Sequence: Synthetic polypeptide"
QVQLVESGGGVVQPGRSLRLSCAASGFTFSSYTMHWVRQAPGKGLEWVTFISYDGNNKYYADSVKGRFTISRDNSKNTLYLQMNSLRAEDTAIYYCARTGWLGPFDYWGQGTLVTVSSASTKGPSVFPLAPSSKSTSGGTAALGCLVKDYFPEPVTVSWNSGALTSGVHTFPAVLQSSGLYSLSSVVTVPSSSLGTQTYICNVNHKPSNTKVDKRVEPKSCDKTHTCPPCPAPELLGGPSVFLFPPKPKDTLMISRTPEVTCVVVDVSHEDPEVKFNWYVDGVEVHNAKTKPREEQYNSTYRVVSVLTVLHQDWLNGKEYKCKVSNKALPAPIEKTISKAKGGGGSGGGPDIQNPDPAVYQLRDSKSSDKSVCLFTDFDSQTNVSQSKDSDVYITDKCVLDMRSMDFKSNSAVAWSNKSDFACANAFNNSIIPEDTFFPSPE

SEQ ID NO: 127 - protein, 443 aa, synthetic construct
  REGION 1..443: note = source = /note="Description of Artificial Sequence: Synthetic polypeptide"
QVQLVESGGGVVQPGRSLRLSCAASGFTFSSYTMHWVRQAPGKGLEWVTFISYDGNNKYYADSVKGRFTISRDNSKNTLYLQMNSLRAEDTAIYYCARTGWLGPFDYWGQGTLVTVSSASTKGPSVFPLAPSSKSTSGGTAALGCLVKDYFPEPVTVSWNSGALTSGVHTFPAVLQSSGLYSLSSVVTVPSSSLGTQTYICNVNHKPSNTKVDKRVEPKSCDKTHTCPPCPAPELLGGPSVFLFPPKPKDTLMISRTPEVTCVVVDVSHEDPEVKFNWYVDGVEVHNAKTKPREEQYNSTYRVVSVLTVLHQDWLNGKEYKCKVSNKALPAPIEKTISKAKGGGGSGGGGPDIQNPDPAVYQLRDSKSSDKSVCLFTDFDSQTNVSQSKDSDVYITDKCVLDMRSMDFKSNSAVAWSNKSDFACANAFNNSIIPEDTFFPSPE

SEQ ID NO: 128 - protein, 444 aa, synthetic construct
  REGION 1..444: note = source = /note="Description of Artificial Sequence: Synthetic polypeptide"
QVQLVESGGGVVQPGRSLRLSCAASGFTFSSYTMHWVRQAPGKGLEWVTFISYDGNNKYYADSVKGRFTISRDNSKNTLYLQMNSLRAEDTAIYYCARTGWLGPFDYWGQGTLVTVSSASTKGPSVFPLAPSSKSTSGGTAALGCLVKDYFPEPVTVSWNSGALTSGVHTFPAVLQSSGLYSLSSVVTVPSSSLGTQTYICNVNHKPSNTKVDKRVEPKSCDKTHTCPPCPAPELLGGPSVFLFPPKPKDTLMISRTPEVTCVVVDVSHEDPEVKFNWYVDGVEVHNAKTKPREEQYNSTYRVVSVLTVLHQDWLNGKEYKCKVSNKALPAPIEKTISKAKGGGGSGGGGSPDIQNPDPAVYQLRDSKSSDKSVCLFTDFDSQTNVSQSKDSDVYITDKCVLDMRSMDFKSNSAVAWSNKSDFACANAFNNSIIPEDTFFPSPE

SEQ ID NO: 129 - protein, 108 aa, synthetic construct; identical to SEQ ID NO: 92
  REGION 1..108: note = source = /note="Description of Artificial Sequence: Synthetic polypeptide"

SEQ ID NO: 130 - protein, 468 aa, synthetic construct
  REGION 1..468: note = source = /note="Description of Artificial Sequence: Synthetic polypeptide"
QVQLVESGGGVVQPGRSLRLSCAASGFTFSSYGMHWVRQAPGKGLEWVAFIRYDGSNKYYADSVKGRFTISRDNSKNTLYLQMNSLRAEDTAVYYCKTHGSHDNWGQGTMVTVSSASTKGPSVFPLAPSSKSTSGGTAALGCLVKDYFPEPVTVSWNSGALTSGVHTFPAVLQSSGLYSLSSVVTVPSSSLGTQTYICNVNHKPSNTKVDKRVEPKSCDKTHTCPPCPAPELLGGPSVFLFPPKPKDTLMISRTPEVTCVVVDVSHEDPEVKFNWYVDGVEVHNAKTKPREEQYNSTYRVVSVLTVLHQDWLNGKEYKCKVSNKALPAPIEKTISKAKEDLNKVFPPEVALFEPSEAEISHTQKATLVCLATGFYPDHVELSWWVNGKEVHSGVCTDPQPLKEQPALNDSRYALSSRLRVSATFWQDPRNHFRCQVQFYGLSEADEWTQARAKPVTQIVSAEAWGRAD

SEQ ID NO: 131 - protein, 469 aa, synthetic construct
  REGION 1..469: note = source = /note="Description of Artificial Sequence: Synthetic polypeptide"
QVQLVESGGGVVQPGRSLRLSCAASGFTFSSYGMHWVRQAPGKGLEWVAFIRYDGSNKYYADSVKGRFTISRDNSKNTLYLQMNSLRAEDTAVYYCKTHGSHDNWGQGTMVTVSSASTKGPSVFPLAPSSKSTSGGTAALGCLVKDYFPEPVTVSWNSGALTSGVHTFPAVLQSSGLYSLSSVVTVPSSSLGTQTYICNVNHKPSNTKVDKRVEPKSCDKTHTCPPCPAPELLGGPSVFLFPPKPKDTLMISRTPEVTCVVVDVSHEDPEVKFNWYVDGVEVHNAKTKPREEQYNSTYRVVSVLTVLHQDWLNGKEYKCKVSNKALPAPIEKTISKAKGEDLNKVFPPEVALFEPSEAEISHTQKATLVCLATGFYPDHVELSWWVNGKEVHSGVCTDPQPLKEQPALNDSRYALSSRLRVSATFWQDPRNHFRCQVQFYGLSEADEWTQARAKPVTQIVSAEAWGRAD

SEQ ID NO: 132 - protein, 470 aa, synthetic construct
  REGION 1..470: note = source = /note="Description of Artificial Sequence: Synthetic polypeptide"
QVQLVESGGGVVQPGRSLRLSCAASGFTFSSYGMHWVRQAPGKGLEWVAFIRYDGSNKYYADSVKGRFTISRDNSKNTLYLQMNSLRAEDTAVYYCKTHGSHDNWGQGTMVTVSSASTKGPSVFPLAPSSKSTSGGTAALGCLVKDYFPEPVTVSWNSGALTSGVHTFPAVLQSSGLYSLSSVVTVPSSSLGTQTYICNVNHKPSNTKVDKRVEPKSCDKTHTCPPCPAPELLGGPSVFLFPPKPKDTLMISRTPEVTCVVVDVSHEDPEVKFNWYVDGVEVHNAKTKPREEQYNSTYRVVSVLTVLHQDWLNGKEYKCKVSNKALPAPIEKTISKAKGGEDLNKVFPPEVALFEPSEAEISHTQKATLVCLATGFYPDHVELSWWVNGKEVHSGVCTDPQPLKEQPALNDSRYALSSRLRVSATFWQDPRNHFRCQVQFYGLSEADEWTQARAKPVTQIVSAEAWGRAD

SEQ ID NO: 133 - protein, 471 aa, synthetic construct
  REGION 1..471: note = source = /note="Description of Artificial Sequence: Synthetic polypeptide"
QVQLVESGGGVVQPGRSLRLSCAASGFTFSSYGMHWVRQAPGKGLEWVAFIRYDGSNKYYADSVKGRFTISRDNSKNTLYLQMNSLRAEDTAVYYCKTHGSHDNWGQGTMVTVSSASTKGPSVFPLAPSSKSTSGGTAALGCLVKDYFPEPVTVSWNSGALTSGVHTFPAVLQSSGLYSLSSVVTVPSSSLGTQTYICNVNHKPSNTKVDKRVEPKSCDKTHTCPPCPAPELLGGPSVFLFPPKPKDTLMISRTPEVTCVVVDVSHEDPEVKFNWYVDGVEVHNAKTKPREEQYNSTYRVVSVLTVLHQDWLNGKEYKCKVSNKALPAPIEKTISKAKGGGEDLNKVFPPEVALFEPSEAEISHTQKATLVCLATGFYPDHVELSWWVNGKEVHSGVCTDPQPLKEQPALNDSRYALSSRLRVSATFWQDPRNHFRCQVQFYGLSEADEWTQARAKPVTQIVSAEAWGRAD

SEQ ID NO: 134 - protein, 472 aa, synthetic construct
  REGION 1..472: note = source = /note="Description of Artificial Sequence: Synthetic polypeptide"
QVQLVESGGGVVQPGRSLRLSCAASGFTFSSYGMHWVRQAPGKGLEWVAFIRYDGSNKYYADSVKGRFTISRDNSKNTLYLQMNSLRAEDTAVYYCKTHGSHDNWGQGTMVTVSSASTKGPSVFPLAPSSKSTSGGTAALGCLVKDYFPEPVTVSWNSGALTSGVHTFPAVLQSSGLYSLSSVVTVPSSSLGTQTYICNVNHKPSNTKVDKRVEPKSCDKTHTCPPCPAPELLGGPSVFLFPPKPKDTLMISRTPEVTCVVVDVSHEDPEVKFNWYVDGVEVHNAKTKPREEQYNSTYRVVSVLTVLHQDWLNGKEYKCKVSNKALPAPIEKTISKAKGGGGEDLNKVFPPEVALFEPSEAEISHTQKATLVCLATGFYPDHVELSWWVNGKEVHSGVCTDPQPLKEQPALNDSRYALSSRLRVSATFWQDPRNHFRCQVQFYGLSEADEWTQARAKPVTQIVSAEAWGRAD

SEQ ID NO: 135 - protein, 473 aa, synthetic construct
  REGION 1..473: note = source = /note="Description of Artificial Sequence: Synthetic polypeptide"
QVQLVESGGGVVQPGRSLRLSCAASGFTFSSYGMHWVRQAPGKGLEWVAFIRYDGSNKYYADSVKGRFTISRDNSKNTLYLQMNSLRAEDTAVYYCKTHGSHDNWGQGTMVTVSSASTKGPSVFPLAPSSKSTSGGTAALGCLVKDYFPEPVTVSWNSGALTSGVHTFPAVLQSSGLYSLSSVVTVPSSSLGTQTYICNVNHKPSNTKVDKRVEPKSCDKTHTCPPCPAPELLGGPSVFLFPPKPKDTLMISRTPEVTCVVVDVSHEDPEVKFNWYVDGVEVHNAKTKPREEQYNSTYRVVSVLTVLHQDWLNGKEYKCKVSNKALPAPIEKTISKAKGGGGSEDLNKVFPPEVALFEPSEAEISHTQKATLVCLATGFYPDHVELSWWVNGKEVHSGVCTDPQPLKEQPALNDSRYALSSRLRVSATFWQDPRNHFRCQVQFYGLSEADEWTQARAKPVTQIVSAEAWGRAD

SEQ ID NO: 136 - protein, 474 aa, synthetic construct
  REGION 1..474: note = source = /note="Description of Artificial Sequence: Synthetic polypeptide"
QVQLVESGGGVVQPGRSLRLSCAASGFTFSSYGMHWVRQAPGKGLEWVAFIRYDGSNKYYADSVKGRFTISRDNSKNTLYLQMNSLRAEDTAVYYCKTHGSHDNWGQGTMVTVSSASTKGPSVFPLAPSSKSTSGGTAALGCLVKDYFPEPVTVSWNSGALTSGVHTFPAVLQSSGLYSLSSVVTVPSSSLGTQTYICNVNHKPSNTKVDKRVEPKSCDKTHTCPPCPAPELLGGPSVFLFPPKPKDTLMISRTPEVTCVVVDVSHEDPEVKFNWYVDGVEVHNAKTKPREEQYNSTYRVVSVLTVLHQDWLNGKEYKCKVSNKALPAPIEKTISKAKGGGGSGEDLNKVFPPEVALFEPSEAEISHTQKATLVCLATGFYPDHVELSWWVNGKEVHSGVCTDPQPLKEQPALNDSRYALSSRLRVSATFWQDPRNHFRCQVQFYGLSEADEWTQARAKPVTQIVSAEAWGRAD

SEQ ID NO: 137 - protein, 475 aa, synthetic construct
  REGION 1..475: note = source = /note="Description of Artificial Sequence: Synthetic polypeptide"
QVQLVESGGGVVQPGRSLRLSCAASGFTFSSYGMHWVRQAPGKGLEWVAFIRYDGSNKYYADSVKGRFTISRDNSKNTLYLQMNSLRAEDTAVYYCKTHGSHDNWGQGTMVTVSSASTKGPSVFPLAPSSKSTSGGTAALGCLVKDYFPEPVTVSWNSGALTSGVHTFPAVLQSSGLYSLSSVVTVPSSSLGTQTYICNVNHKPSNTKVDKRVEPKSCDKTHTCPPCPAPELLGGPSVFLFPPKPKDTLMISRTPEVTCVVVDVSHEDPEVKFNWYVDGVEVHNAKTKPREEQYNSTYRVVSVLTVLHQDWLNGKEYKCKVSNKALPAPIEKTISKAKGGGGSGGEDLNKVFPPEVALFEPSEAEISHTQKATLVCLATGFYPDHVELSWWVNGKEVHSGVCTDPQPLKEQPALNDSRYALSSRLRVSATFWQDPRNHFRCQVQFYGLSEADEWTQARAKPVTQIVSAEAWGRAD

SEQ ID NO: 138 - protein, 476 aa, synthetic construct
  REGION 1..476: note = source = /note="Description of Artificial Sequence: Synthetic polypeptide"
QVQLVESGGGVVQPGRSLRLSCAASGFTFSSYGMHWVRQAPGKGLEWVAFIRYDGSNKYYADSVKGRFTISRDNSKNTLYLQMNSLRAEDTAVYYCKTHGSHDNWGQGTMVTVSSASTKGPSVFPLAPSSKSTSGGTAALGCLVKDYFPEPVTVSWNSGALTSGVHTFPAVLQSSGLYSLSSVVTVPSSSLGTQTYICNVNHKPSNTKVDKRVEPKSCDKTHTCPPCPAPELLGGPSVFLFPPKPKDTLMISRTPEVTCVVVDVSHEDPEVKFNWYVDGVEVHNAKTKPREEQYNSTYRVVSVLTVLHQDWLNGKEYKCKVSNKALPAPIEKTISKAKGGGGSGGGEDLNKVFPPEVALFEPSEAEISHTQKATLVCLATGFYPDHVELSWWVNGKEVHSGVCTDPQPLKEQPALNDSRYALSSRLRVSATFWQDPRNHFRCQVQFYGLSEADEWTQARAKPVTQIVSAEAWGRAD

SEQ ID NO: 139 - protein, 477 aa, synthetic construct
  REGION 1..477: note = source = /note="Description of Artificial Sequence: Synthetic polypeptide"
QVQLVESGGGVVQPGRSLRLSCAASGFTFSSYGMHWVRQAPGKGLEWVAFIRYDGSNKYYADSVKGRFTISRDNSKNTLYLQMNSLRAEDTAVYYCKTHGSHDNWGQGTMVTVSSASTKGPSVFPLAPSSKSTSGGTAALGCLVKDYFPEPVTVSWNSGALTSGVHTFPAVLQSSGLYSLSSVVTVPSSSLGTQTYICNVNHKPSNTKVDKRVEPKSCDKTHTCPPCPAPELLGGPSVFLFPPKPKDTLMISRTPEVTCVVVDVSHEDPEVKFNWYVDGVEVHNAKTKPREEQYNSTYRVVSVLTVLHQDWLNGKEYKCKVSNKALPAPIEKTISKAKGGGGSGGGGEDLNKVFPPEVALFEPSEAEISHTQKATLVCLATGFYPDHVELSWWVNGKEVHSGVCTDPQPLKEQPALNDSRYALSSRLRVSATFWQDPRNHFRCQVQFYGLSEADEWTQARAKPVTQIVSAEAWGRAD

SEQ ID NO: 140 - protein, 478 aa, synthetic construct
  REGION 1..478: note = source = /note="Description of Artificial Sequence: Synthetic polypeptide"
QVQLVESGGGVVQPGRSLRLSCAASGFTFSSYGMHWVRQAPGKGLEWVAFIRYDGSNKYYADSVKGRFTISRDNSKNTLYLQMNSLRAEDTAVYYCKTHGSHDNWGQGTMVTVSSASTKGPSVFPLAPSSKSTSGGTAALGCLVKDYFPEPVTVSWNSGALTSGVHTFPAVLQSSGLYSLSSVVTVPSSSLGTQTYICNVNHKPSNTKVDKRVEPKSCDKTHTCPPCPAPELLGGPSVFLFPPKPKDTLMISRTPEVTCVVVDVSHEDPEVKFNWYVDGVEVHNAKTKPREEQYNSTYRVVSVLTVLHQDWLNGKEYKCKVSNKALPAPIEKTISKAKGGGGSGGGGSEDLNKVFPPEVALFEPSEAEISHTQKATLVCLATGFYPDHVELSWWVNGKEVHSGVCTDPQPLKEQPALNDSRYALSSRLRVSATFWQDPRNHFRCQVQFYGLSEADEWTQARAKPVTQIVSAEAWGRAD

SEQ ID NO: 141 - protein, 217 aa, synthetic construct
  REGION 1..217: note = source = /note="Description of Artificial Sequence: Synthetic polypeptide"
QSVLTQPPSVSGAPGQRVTISCSGSRSNIGSNTVKWYQQLPGTAPKLLIYYNDQRPSGVPDRFSGSKSGTSASLAITGLQAEDEADYYCQSYDRYTHPALLFGTGTKVTVLGQPKANPTVTLFPPSSEELQANKATLVCLISDFYPGAVTVAWKADGSPVKAGVETTKPSKQSNNKYAASSYLSLTPEQWKSHRSYSCQVTHEGSTVEKTVAPTECS

SEQ ID NO: 142 - protein, 234 aa, synthetic construct
  REGION 1..234: note = source = /note="Description of Artificial Sequence: Synthetic polypeptide"
TIKPCPPCKCPAPNLLGGPSVFIFPPKIKDVLMISLSPIVTCVVVDVSEDDPDVQISWFVNNVEVHTAQTQTHREDYNSTLRVVSALPIQHQDWMSGKEFKCKVNNKDLPAPIERTISKPKPNIQNPEPAVYQLKDPRSQDSTLCLFTDFDSQINVPKTMESGTFITDKCVLDMKAMDSKSNGAIAWSNQTSFTCQDIFKETNATYPSSDVPCDATLTEKSFETDMNLNFQNLS

SEQ ID NO: 143 - protein, 235 aa, synthetic construct
  REGION 1..235: note = source = /note="Description of Artificial Sequence: Synthetic polypeptide"
TIKPCPPCKCPAPNLLGGPSVFIFPPKIKDVLMISLSPIVTCVVVDVSEDDPDVQISWFVNNVEVHTAQTQTHREDYNSTLRVVSALPIQHQDWMSGKEFKCKVNNKDLPAPIERTISKPGKPNIQNPEPAVYQLKDPRSQDSTLCLFTDFDSQINVPKTMESGTFITDKCVLDMKAMDSKSNGAIAWSNQTSFTCQDIFKETNATYPSSDVPCDATLTEKSFETDMNLNFQNLS

SEQ ID NO: 144 - protein, 236 aa, synthetic construct
  REGION 1..236: note = source = /note="Description of Artificial Sequence: Synthetic polypeptide"
TIKPCPPCKCPAPNLLGGPSVFIFPPKIKDVLMISLSPIVTCVVVDVSEDDPDVQISWFVNNVEVHTAQTQTHREDYNSTLRVVSALPIQHQDWMSGKEFKCKVNNKDLPAPIERTISKPGGKPNIQNPEPAVYQLKDPRSQDSTLCLFTDFDSQINVPKTMESGTFITDKCVLDMKAMDSKSNGAIAWSNQTSFTCQDIFKETNATYPSSDVPCDATLTEKSFETDMNLNFQNLS

SEQ ID NO: 145 - protein, 237 aa, synthetic construct
  REGION 1..237: note = source = /note="Description of Artificial Sequence: Synthetic polypeptide"
TIKPCPPCKCPAPNLLGGPSVFIFPPKIKDVLMISLSPIVTCVVVDVSEDDPDVQISWFVNNVEVHTAQTQTHREDYNSTLRVVSALPIQHQDWMSGKEFKCKVNNKDLPAPIERTISKPGGGKPNIQNPEPAVYQLKDPRSQDSTLCLFTDFDSQINVPKTMESGTFITDKCVLDMKAMDSKSNGAIAWSNQTSFTCQDIFKETNATYPSSDVPCDATLTEKSFETDMNLNFQNLS

SEQ ID NO: 146 - protein, 238 aa, synthetic construct
  REGION 1..238: note = source = /note="Description of Artificial Sequence: Synthetic polypeptide"
TIKPCPPCKCPAPNLLGGPSVFIFPPKIKDVLMISLSPIVTCVVVDVSEDDPDVQISWFVNNVEVHTAQTQTHREDYNSTLRVVSALPIQHQDWMSGKEFKCKVNNKDLPAPIERTISKPGGGGKPNIQNPEPAVYQLKDPRSQDSTLCLFTDFDSQINVPKTMESGTFITDKCVLDMKAMDSKSNGAIAWSNQTSFTCQDIFKETNATYPSSDVPCDATLTEKSFETDMNLNFQNLS

SEQ ID NO: 147 - protein, 239 aa, synthetic construct
  REGION 1..239: note = source = /note="Description of Artificial Sequence: Synthetic polypeptide"
TIKPCPPCKCPAPNLLGGPSVFIFPPKIKDVLMISLSPIVTCVVVDVSEDDPDVQISWFVNNVEVHTAQTQTHREDYNSTLRVVSALPIQHQDWMSGKEFKCKVNNKDLPAPIERTISKPGGGGSKPNIQNPEPAVYQLKDPRSQDSTLCLFTDFDSQINVPKTMESGTFITDKCVLDMKAMDSKSNGAIAWSNQTSFTCQDIFKETNATYPSSDVPCDATLTEKSFETDMNLNFQNLS

SEQ ID NO: 148 - protein, 240 aa, synthetic construct
  REGION 1..240: note = source = /note="Description of Artificial Sequence: Synthetic polypeptide"
TIKPCPPCKCPAPNLLGGPSVFIFPPKIKDVLMISLSPIVTCVVVDVSEDDPDVQISWFVNNVEVHTAQTQTHREDYNSTLRVVSALPIQHQDWMSGKEFKCKVNNKDLPAPIERTISKPGGGGSGKPNIQNPEPAVYQLKDPRSQDSTLCLFTDFDSQINVPKTMESGTFITDKCVLDMKAMDSKSNGAIAWSNQTSFTCQDIFKETNATYPSSDVPCDATLTEKSFETDMNLNFQNLS

SEQ ID NO: 149 - protein, 241 aa, synthetic construct
  REGION 1..241: note = source = /note="Description of Artificial Sequence: Synthetic polypeptide"
TIKPCPPCKCPAPNLLGGPSVFIFPPKIKDVLMISLSPIVTCVVVDVSEDDPDVQISWFVNNVEVHTAQTQTHREDYNSTLRVVSALPIQHQDWMSGKEFKCKVNNKDLPAPIERTISKPGGGGSGGKPNIQNPEPAVYQLKDPRSQDSTLCLFTDFDSQINVPKTMESGTFITDKCVLDMKAMDSKSNGAIAWSNQTSFTCQDIFKETNATYPSSDVPCDATLTEKSFETDMNLNFQNLS

SEQ ID NO: 150 - protein, 242 aa, synthetic construct
  REGION 1..242: note = source = /note="Description of Artificial Sequence: Synthetic polypeptide"
TIKPCPPCKCPAPNLLGGPSVFIFPPKIKDVLMISLSPIVTCVVVDVSEDDPDVQISWFVNNVEVHTAQTQTHREDYNSTLRVVSALPIQHQDWMSGKEFKCKVNNKDLPAPIERTISKPGGGGSGGGKPNIQNPEPAVYQLKDPRSQDSTLCLFTDFDSQINVPKTMESGTFITDKCVLDMKAMDSKSNGAIAWSNQTSFTCQDIFKETNATYPSSDVPCDATLTEKSFETDMNLNFQNLS

SEQ ID NO: 151 - protein, 243 aa, synthetic construct
  REGION 1..243: note = source = /note="Description of Artificial Sequence: Synthetic polypeptide"
TIKPCPPCKCPAPNLLGGPSVFIFPPKIKDVLMISLSPIVTCVVVDVSEDDPDVQISWFVNNVEVHTAQTQTHREDYNSTLRVVSALPIQHQDWMSGKEFKCKVNNKDLPAPIERTISKPGGGGSGGGGKPNIQNPEPAVYQLKDPRSQDSTLCLFTDFDSQINVPKTMESGTFITDKCVLDMKAMDSKSNGAIAWSNQTSFTCQDIFKETNATYPSSDVPCDATLTEKSFETDMNLNFQNLS

SEQ ID NO: 152 - protein, 244 aa, synthetic construct
  REGION 1..244: note = source = /note="Description of Artificial Sequence: Synthetic polypeptide"
TIKPCPPCKCPAPNLLGGPSVFIFPPKIKDVLMISLSPIVTCVVVDVSEDDPDVQISWFVNNVEVHTAQTQTHREDYNSTLRVVSALPIQHQDWMSGKEFKCKVNNKDLPAPIERTISKPGGGGSGGGGSKPNIQNPEPAVYQLKDPRSQDSTLCLFTDFDSQINVPKTMESGTFITDKCVLDMKAMDSKSNGAIAWSNQTSFTCQDIFKETNATYPSSDVPCDATLTEKSFETDMNLNFQNLS

SEQ ID NO: 153 - protein, 387 aa, synthetic construct
  REGION 1..387: note = source = /note="Description of Artificial Sequence: Synthetic polypeptide"
TIKPCPPCKCPAPNLLGGPSVFIFPPKIKDVLMISLSPIVTCVVVDVSEDDPDVQISWFVNNVEVHTAQTQTHREDYNSTLRVVSALPIQHQDWMSGKEFKCKVNNKDLPAPIERTISKPVVEDLRNVTPPKVSLFEPSKAEIANKQKATLVCLARGFFPDHVELSWWVNGKEVHSGVCTDPQAYKESNYSYSLSSRLRVSATFWHNPRNHFRCQVQFHGLSEEDKWPEGSPKPVTQNISAEAWGRADGGGGSGGGGSGGGGSSHLEQLLMDLQELLSRMENYRNLKLPRMLTAKFALPKQATELKDLQCLEDELGPLRHVLDLTQSKSFQLEDAENFISNIRVTVVKLKGSDNTFECQFDDESATVVDFLRRWIAFCQSIISTSPQ

SEQ ID NO: 154 - protein, 388 aa, synthetic construct
  REGION 1..388: note = source = /note="Description of Artificial Sequence: Synthetic polypeptide"
TIKPCPPCKCPAPNLLGGPSVFIFPPKIKDVLMISLSPIVTCVVVDVSEDDPDVQISWFVNNVEVHTAQTQTHREDYNSTLRVVSALPIQHQDWMSGKEFKCKVNNKDLPAPIERTISKPGVVEDLRNVTPPKVSLFEPSKAEIANKQKATLVCLARGFFPDHVELSWWVNGKEVHSGVCTDPQAYKESNYSYSLSSRLRVSATFWHNPRNHFRCQVQFHGLSEEDKWPEGSPKPVTQNISAEAWGRADGGGGSGGGGSGGGGSSHLEQLLMDLQELLSRMENYRNLKLPRMLTAKFALPKQATELKDLQCLEDELGPLRHVLDLTQSKSFQLEDAENFISNIRVTVVKLKGSDNTFECQFDDESATVVDFLRRWIAFCQSIISTSPQ

SEQ ID NO: 155 - protein, 389 aa, synthetic construct
  REGION 1..389: note = source = /note="Description of Artificial Sequence: Synthetic polypeptide"
TIKPCPPCKCPAPNLLGGPSVFIFPPKIKDVLMISLSPIVTCVVVDVSEDDPDVQISWFVNNVEVHTAQTQTHREDYNSTLRVVSALPIQHQDWMSGKEFKCKVNNKDLPAPIERTISKPGGVVEDLRNVTPPKVSLFEPSKAEIANKQKATLVCLARGFFPDHVELSWWVNGKEVHSGVCTDPQAYKESNYSYSLSSRLRVSATFWHNPRNHFRCQVQFHGLSEEDKWPEGSPKPVTQNISAEAWGRADGGGGSGGGGSGGGGSSHLEQLLMDLQELLSRMENYRNLKLPRMLTAKFALPKQATELKDLQCLEDELGPLRHVLDLTQSKSFQLEDAENFISNIRVTVVKLKGSDNTFECQFDDESATVVDFLRRWIAFCQSIISTSPQ

SEQ ID NO: 156 - protein, 390 aa, synthetic construct
  REGION 1..390: note = source = /note="Description of Artificial Sequence: Synthetic polypeptide"
TIKPCPPCKCPAPNLLGGPSVFIFPPKIKDVLMISLSPIVTCVVVDVSEDDPDVQISWFVNNVEVHTAQTQTHREDYNSTLRVVSALPIQHQDWMSGKEFKCKVNNKDLPAPIERTISKPGGGVVEDLRNVTPPKVSLFEPSKAEIANKQKATLVCLARGFFPDHVELSWWVNGKEVHSGVCTDPQAYKESNYSYSLSSRLRVSATFWHNPRNHFRCQVQFHGLSEEDKWPEGSPKPVTQNISAEAWGRADGGGGSGGGGSGGGGSSHLEQLLMDLQELLSRMENYRNLKLPRMLTAKFALPKQATELKDLQCLEDELGPLRHVLDLTQSKSFQLEDAENFISNIRVTVVKLKGSDNTFECQFDDESATVVDFLRRWIAFCQSIISTSPQ

SEQ ID NO: 157 - protein, 391 aa, synthetic construct
  REGION 1..391: note = source = /note="Description of Artificial Sequence: Synthetic polypeptide"
TIKPCPPCKCPAPNLLGGPSVFIFPPKIKDVLMISLSPIVTCVVVDVSEDDPDVQISWFVNNVEVHTAQTQTHREDYNSTLRVVSALPIQHQDWMSGKEFKCKVNNKDLPAPIERTISKPGGGGVVEDLRNVTPPKVSLFEPSKAEIANKQKATLVCLARGFFPDHVELSWWVNGKEVHSGVCTDPQAYKESNYSYSLSSRLRVSATFWHNPRNHFRCQVQFHGLSEEDKWPEGSPKPVTQNISAEAWGRADGGGGSGGGGSGGGGSSHLEQLLMDLQELLSRMENYRNLKLPRMLTAKFALPKQATELKDLQCLEDELGPLRHVLDLTQSKSFQLEDAENFISNIRVTVVKLKGSDNTFECQFDDESATVVDFLRRWIAFCQSIISTSPQ

SEQ ID NO: 158 - protein, 142 aa, Homo sapiens
PNIQNPDPAVYQLRDSKSSDKSVCLFTDFDSQTNVSQSKDSDVYITDKTVLDMRSMDFKSNSAVAWSNKSDFACANAFNNSIIPEDTFFPSPESSCDVKLVEKSFETDTNLNFQNLSVIGFRILLLKVAGFNLLMTLRLWSS

SEQ ID NO: 159 - protein, 177 aa, Homo sapiens
EDLNKVFPPEVAVFEPSEAEISHTQKATLVCLATGFFPDHVELSWWVNGKEVHSGVSTDPQPLKEQPALNDSRYCLSSRLRVSATFWQNPRNHFRCQVQFYGLSENDEWTQDRAKPVTQIVSAEAWGRADCGFTSVSYQQGVLSATILYEILLGKATLYAVLVSALVLMAMVKRKDF

SEQ ID NO: 160 - protein, 394 aa, synthetic construct
  REGION 1..394: note = source = /note="Description of Artificial Sequence: Synthetic polypeptide"
TIKPCPPCKCPAPNLLGGPSVFIFPPKIKDVLMISLSPIVTCVVVDVSEDDPDVQISWFVNNVEVHTAQTQTHREDYNSTLRVVSALPIQHQDWMSGKEFKCKVNNKDLPAPIERTISKPGGGGSGGVVEDLRNVTPPKVSLFEPSKAEIANKQKATLVCLARGFFPDHVELSWWVNGKEVHSGVCTDPQAYKESNYSYSLSSRLRVSATFWHNPRNHFRCQVQFHGLSEEDKWPEGSPKPVTQNISAEAWGRADGGGGSGGGGSGGGGSSHLEQLLMDLQELLSRMENYRNLKLPRMLTAKFALPKQATELKDLQCLEDELGPLRHVLDLTQSKSFQLEDAENFISNIRVTVVKLKGSDNTFECQFDDESATVVDFLRRWIAFCQSIISTSPQ

SEQ ID NO: 161 - protein, 395 aa, synthetic construct
  REGION 1..395: note = source = /note="Description of Artificial Sequence: Synthetic polypeptide"
TIKPCPPCKCPAPNLLGGPSVFIFPPKIKDVLMISLSPIVTCVVVDVSEDDPDVQISWFVNNVEVHTAQTQTHREDYNSTLRVVSALPIQHQDWMSGKEFKCKVNNKDLPAPIERTISKPGGGGSGGGVVEDLRNVTPPKVSLFEPSKAEIANKQKATLVCLARGFFPDHVELSWWVNGKEVHSGVCTDPQAYKESNYSYSLSSRLRVSATFWHNPRNHFRCQVQFHGLSEEDKWPEGSPKPVTQNISAEAWGRADGGGGSGGGGSGGGGSSHLEQLLMDLQELLSRMENYRNLKLPRMLTAKFALPKQATELKDLQCLEDELGPLRHVLDLTQSKSFQLEDAENFISNIRVTVVKLKGSDNTFECQFDDESATVVDFLRRWIAFCQSIISTSPQ

SEQ ID NO: 162 - protein, 396 aa, synthetic construct
  REGION 1..396: note = source = /note="Description of Artificial Sequence: Synthetic polypeptide"
TIKPCPPCKCPAPNLLGGPSVFIFPPKIKDVLMISLSPIVTCVVVDVSEDDPDVQISWFVNNVEVHTAQTQTHREDYNSTLRVVSALPIQHQDWMSGKEFKCKVNNKDLPAPIERTISKPGGGGSGGGGVVEDLRNVTPPKVSLFEPSKAEIANKQKATLVCLARGFFPDHVELSWWVNGKEVHSGVCTDPQAYKESNYSYSLSSRLRVSATFWHNPRNHFRCQVQFHGLSEEDKWPEGSPKPVTQNISAEAWGRADGGGGSGGGGSGGGGSSHLEQLLMDLQELLSRMENYRNLKLPRMLTAKFALPKQATELKDLQCLEDELGPLRHVLDLTQSKSFQLEDAENFISNIRVTVVKLKGSDNTFECQFDDESATVVDFLRRWIAFCQSIISTSPQ

SEQ ID NO: 163 - protein, 397 aa, synthetic construct
  REGION 1..397: note = source = /note="Description of Artificial Sequence: Synthetic polypeptide"
TIKPCPPCKCPAPNLLGGPSVFIFPPKIKDVLMISLSPIVTCVVVDVSEDDPDVQISWFVNNVEVHTAQTQTHREDYNSTLRVVSALPIQHQDWMSGKEFKCKVNNKDLPAPIERTISKPGGGGSGGGGSVVEDLRNVTPPKVSLFEPSKAEIANKQKATLVCLARGFFPDHVELSWWVNGKEVHSGVCTDPQAYKESNYSYSLSSRLRVSATFWHNPRNHFRCQVQFHGLSEEDKWPEGSPKPVTQNISAEAWGRADGGGGSGGGGSGGGGSSHLEQLLMDLQELLSRMENYRNLKLPRMLTAKFALPKQATELKDLQCLEDELGPLRHVLDLTQSKSFQLEDAENFISNIRVTVVKLKGSDNTFECQFDDESATVVDFLRRWIAFCQSIISTSPQ

SEQ ID NO: 164 - protein, 448 aa, synthetic construct
  REGION 1..448: note = source = /note="Description of Artificial Sequence: Synthetic polypeptide"
QVQLVESGGGVVQPGRSLRLSCAASGFTFSSYTMHWVRQAPGKGLEWVTFISYDGNNKYYADSVKGRFTISRDNSKNTLYLQMNSLRAEDTAIYYCARTGWLGPFDYWGQGTLVTVSSASTKGPSVFPLAPSSKSTSGGTAALGCLVKDYFPEPVTVSWNSGALTSGVHTFPAVLQSSGLYSLSSVVTVPSSSLGTQTYICNVNHKPSNTKVDKRVEPKSCDKTHTCPPCPAPELLGGPSVFLFPPKPKDTLMISRTPEVTCVVVDVSHEDPEVKFNWYVDGVEVHNAKTKPREEQYNSTYRVVSVLTVLHQDWLNGKEYKCKVSNKALPAPIEKTISKAKGQPREPQVYTLPPCREEMTKNQVSLWCLVKGFYPSDIAVEWESNGQPENNYKTTPPVLDSDGSFFLYSKLTVDKSRWQQGNVFSCSVMHEALHNHYTQKSLSLSPGK

SEQ ID NO: 165 - protein, 445 aa, synthetic construct
  REGION 1..445: note = source = /note="Description of Artificial Sequence: Synthetic polypeptide"
QVQLVESGGGVVQPGRSLRLSCAASGFTFSSYGMHWVRQAPGKGLEWVAFIRYDGSNKYYADSVKGRFTISRDNSKNTLYLQMNSLRAEDTAVYYCKTHGSHDNWGQGTMVTVSSASTKGPSVFPLAPSSKSTSGGTAALGCLVKDYFPEPVTVSWNSGALTSGVHTFPAVLQSSGLYSLSSVVTVPSSSLGTQTYICNVNHKPSNTKVDKRVEPKSCDKTHTCPPCPAPELLGGPSVFLFPPKPKDTLMISRTPEVTCVVVDVSHEDPEVKFNWYVDGVEVHNAKTKPREEQYNSTYRVVSVLTVLHQDWLNGKEYKCKVSNKALPAPIEKTISKAKGQPREPQVCTLPPSREEMTKNQVSLSCAVKGFYPSDIAVEWESNGQPENNYKTTPPVLDSDGSFFLVSKLTVDKSRWQQGNVFSCSVMHEALHNHYTQKSLSLSPGK

SEQ ID NO: 166 - protein, 392 aa, synthetic construct
  REGION 1..392: note = source = /note="Description of Artificial Sequence: Synthetic polypeptide"
TIKPCPPCKCPAPNLLGGPSVFIFPPKIKDVLMISLSPIVTCVVVDVSEDDPDVQISWFVNNVEVHTAQTQTHREDYNSTLRVVSALPIQHQDWMSGKEFKCKVNNKDLPAPIERTISKPGGGGSVVEDLRNVTPPKVSLFEPSKAEIANKQKATLVCLARGFFPDHVELSWWVNGKEVHSGVCTDPQAYKESNYSYSLSSRLRVSATFWHNPRNHFRCQVQFHGLSEEDKWPEGSPKPVTQNISAEAWGRADGGGGSGGGGSGGGGSSHLEQLLMDLQELLSRMENYRNLKLPRMLTAKFALPKQATELKDLQCLEDELGPLRHVLDLTQSKSFQLEDAENFISNIRVTVVKLKGSDNTFECQFDDESATVVDFLRRWIAFCQSIISTSPQ

SEQ ID NO: 167 - protein, 393 aa, synthetic construct
  REGION 1..393: note = source = /note="Description of Artificial Sequence: Synthetic polypeptide"
TIKPCPPCKCPAPNLLGGPSVFIFPPKIKDVLMISLSPIVTCVVVDVSEDDPDVQISWFVNNVEVHTAQTQTHREDYNSTLRVVSALPIQHQDWMSGKEFKCKVNNKDLPAPIERTISKPGGGGSGVVEDLRNVTPPKVSLFEPSKAEIANKQKATLVCLARGFFPDHVELSWWVNGKEVHSGVCTDPQAYKESNYSYSLSSRLRVSATFWHNPRNHFRCQVQFHGLSEEDKWPEGSPKPVTQNISAEAWGRADGGGGSGGGGSGGGGSSHLEQLLMDLQELLSRMENYRNLKLPRMLTAKFALPKQATELKDLQCLEDELGPLRHVLDLTQSKSFQLEDAENFISNIRVTVVKLKGSDNTFECQFDDESATVVDFLRRWIAFCQSIISTSPQ

SEQ ID NO: 168 - protein, 90 aa, synthetic construct
  REGION 1..90: note = source = /note="Description of Artificial Sequence: Synthetic polypeptide"
PNIQNPDPAVYQLRDSKSSDKSVCLFTDFDSQTNVSQSKDSDVYITDKTVLDMRSMDFKSNSAVAWSNKFACANAFNNSIIPEDTFFPSP

SEQ ID NO: 169 - protein, 102 aa, synthetic construct
  REGION 1..102: note = source = /note="Description of Artificial Sequence: Synthetic polypeptide"
GQPREPQVYTLPPCRDELTKNQVSLWCLVKGFYPSDIAVEWESNGQPENNYKTTPPVLDSDGSFFLYSKLTVDKSRWQQGNVFSCSVMHEALHNHYTQKSLS

SEQ ID NO: 170 - protein, 129 aa, synthetic construct
  REGION 1..129: note = source = /note="Description of Artificial Sequence: Synthetic polypeptide"
EDLKNVFPPEVAVFEPSEAEISHTQKATLVCLATGFYPDHVELSWWVNGKEVHSGVSTDPQPLKEQPALNDSRYALSSRLRVSATFWQNPRNHFRCQVQFYGLSENDEWTQDRAKPVTQIVSAEAWGRA

SEQ ID NO: 171 - protein, 102 aa, synthetic construct
  REGION 1..102: note = source = /note="Description of Artificial Sequence: Synthetic polypeptide"
GQPREPQVCTLPPSRDELTKNQVSLSCAVKGFYPSDIAVEWESNGQPENNYKTTPPVLDSDGSFFLVSKLTVDKSRWQQGNVFSCSVMHEALHNHYTQKSLS